European Patent Application EP 4 212 631 A1, published July 19, 2023. Title: COMPOSITIONS AND METHODS FOR IMMUNE REPERTOIRE SEQUENCING. Applicant: LIFE TECHNOLOGIES CORPORATION. Application PCT/US2018/049259. The sequence listing filed with the application follows.

SEQUENCE LISTING (505 sequences)

SEQ ID NO: 1 - DNA, 25 bp, Artificial Sequence
  source: /note="Description of Artificial Sequence: Synthetic primer"
aaaatacctggtcacacagacggga

SEQ ID NO: 2 - DNA, 25 bp, Artificial Sequence
  source: /note="Description of Artificial Sequence: Synthetic primer"
aagataccgggttacccagtttgga

SEQ ID NO: 3 - DNA, 30 bp, Artificial Sequence
  source: /note="Description of Artificial Sequence: Synthetic primer"
actcaaactccaagacatctgatcaaaacg

SEQ ID NO: 4 - DNA, 25 bp, Artificial Sequence
  source: /note="Description of Artificial Sequence: Synthetic primer"
agaatcccagacacaagatcacaaa

SEQ ID NO: 5 - DNA, 25 bp, Artificial Sequence
  source: /note="Description of Artificial Sequence: Synthetic primer"
agagtccaagacacaagatcacaga

SEQ ID NO: 6 - DNA, 25 bp, Artificial Sequence
  source: /note="Description of Artificial Sequence: Synthetic primer"
agtccccaagacatctgatcagaga

SEQ ID NO: 7 - DNA, 21 bp, Artificial Sequence
  source: /note="Description of Artificial Sequence: Synthetic primer"
atcaatggccagcgaccctgg

SEQ ID NO: 8 - DNA, 25 bp, Artificial Sequence
  source: /note="Description of Artificial Sequence: Synthetic primer"
ccaaagtcccacacacctgatcaaa

SEQ ID NO: 9 - DNA, 21 bp, Artificial Sequence
  source: /note="Description of Artificial Sequence: Synthetic primer"
cccagacaccaaaatacctgg

SEQ ID NO: 10 - DNA, 27 bp, Artificial Sequence
  source: /note="Description of Artificial Sequence: Synthetic primer"
ctcaacatccgagtagggttatctgta

SEQ ID NO: 11 - DNA, 21 bp, Artificial Sequence
  source: /note="Description of Artificial Sequence: Synthetic primer"
ctcagtccccaaagtacctgt

SEQ ID NO: 12 - DNA, 19 bp, Artificial Sequence
  source: /note="Description of Artificial Sequence: Synthetic primer"
ctggaatcacccagagccc

SEQ ID NO: 13 - DNA, 19 bp, Artificial Sequence
  source: /note="Description of Artificial Sequence: Synthetic primer"
ctggagtctcccacaaccc

SEQ ID NO: 14 - DNA, 19 bp, Artificial Sequence
  source: /note="Description of Artificial Sequence: Synthetic primer"
ctggagtctcccagaaccc

SEQ ID NO: 15 - DNA, 19 bp, Artificial Sequence
  source: /note="Description of Artificial Sequence: Synthetic primer"
ctggagtctcccaggaccc

SEQ ID NO: 16 - DNA, 28 bp, Artificial Sequence
  source: /note="Description of Artificial Sequence: Synthetic primer"
ctggagtcactcaaactccaagatatct

SEQ ID NO: 17 - DNA, 22 bp, Artificial Sequence
  source: /note="Description of Artificial Sequence: Synthetic primer"
gaaagccagtgaccctgagttg

SEQ ID NO: 18 - DNA, 25 bp, Artificial Sequence
  source: /note="Description of Artificial Sequence: Synthetic primer"
cccagagctcgagatatctagtcaa

SEQ ID NO: 19 - DNA, 24 bp, Artificial Sequence
  source: /note="Description of Artificial Sequence: Synthetic primer"
aaaagccaagcagggatatctgtc

SEQ ID NO: 20 - DNA, 25 bp, Artificial Sequence
  source: /note="Description of Artificial Sequence: Synthetic primer"
aaaatacctggtcacacagatggga

SEQ ID NO: 21 - DNA, 24 bp, Artificial Sequence
  source: /note="Description of Artificial Sequence: Synthetic primer"
aaaattccacgtcctgaagacagg

SEQ ID NO: 22 - DNA, 24 bp, Artificial Sequence
  source: /note="Description of Artificial Sequence: Synthetic primer"
aaaattccaggtcctgaagacagg

SEQ ID NO: 23 - DNA, 26 bp, Artificial Sequence
  source: /note="Description of Artificial Sequence: Synthetic primer"
aaaattccacatcctgaagacaggac

SEQ ID NO: 24 - DNA, 23 bp, Artificial Sequence
  source: /note="Description of Artificial Sequence: Synthetic primer"
aaagcacctgatcacagcaactg

SEQ ID NO: 25 - DNA, 24 bp, Artificial Sequence
  source: /note="Description of Artificial Sequence: Synthetic primer"
aacatccgagcagggttatctgta

SEQ ID NO: 26 - DNA, 24 bp, Artificial Sequence
  source: /note="Description of Artificial Sequence: Synthetic primer"
aacatccgagctgggttatctgta

SEQ ID NO: 27 - DNA, 26 bp, Artificial Sequence
  source: /note="Description of Artificial Sequence: Synthetic primer"
aacccaagatacctcatcacagtgac

SEQ ID NO: 28 - DNA, 24 bp, Artificial Sequence
  source: /note="Description of Artificial Sequence: Synthetic primer"
aagacacagaatcattgggacagg

SEQ ID NO: 29 - DNA, 24 bp, Artificial Sequence
  source: /note="Description of Artificial Sequence: Synthetic primer"
aagcatgaggtgacagaaatggga

SEQ ID NO: 30 - DNA, 22 bp, Artificial Sequence
  source: /note="Description of Artificial Sequence: Synthetic primer"
aaggcacaaggtgacagagatg

SEQ ID NO: 31 - DNA, 24 bp, Artificial Sequence
  source: /note="Description of Artificial Sequence: Synthetic primer"
aatacctggtcacacagatgggaa

SEQ ID NO: 32 - DNA, 29 bp, Artificial Sequence
  source: /note="Description of Artificial Sequence: Synthetic primer"
aattctcaagacacagaatcattgggaca

SEQ ID NO: 33 - DNA, 25 bp, Artificial Sequence
  source: /note="Description of Artificial Sequence: Synthetic primer"
acaaagtcccacacacctgatcaaa

SEQ ID NO: 34 - DNA, 21 bp, Artificial Sequence
  source: /note="Description of Artificial Sequence: Synthetic primer"
acacaaggtcaccaacatggg

SEQ ID NO: 35 - DNA, 21 bp, Artificial Sequence
  source: /note="Description of Artificial Sequence: Synthetic primer"
acaccaagacacctggtcatg

SEQ ID NO: 36 - DNA, 22 bp, Artificial Sequence
  source: /note="Description of Artificial Sequence: Synthetic primer"
accaacatctcagatcctggca

SEQ ID NO: 37 - DNA, 26 bp, Artificial Sequence
  source: /note="Description of Artificial Sequence: Synthetic primer"
accagaccccaagataccttgttata

SEQ ID NO: 38 - DNA, 25 bp, Artificial Sequence
  source: /note="Description of Artificial Sequence: Synthetic primer"
accccaaggaataggatcacaaaga

SEQ ID NO: 39 - DNA, 21 bp, Artificial Sequence
  source: /note="Description of Artificial Sequence: Synthetic primer"
acccccagtaacaaggtcaca

SEQ ID NO: 40 - DNA, 26 bp, Artificial Sequence
  source: /note="Description of Artificial Sequence: Synthetic primer"
acctagacttctggtcaaagcaagtg

SEQ ID NO: 41 - DNA, 27 bp, Artificial Sequence
  source: /note="Description of Artificial Sequence: Synthetic primer"
acctagatttctggtcaaagcaaatga

SEQ ID NO: 42 - DNA, 31 bp, Artificial Sequence
  source: /note="Description of Artificial Sequence: Synthetic primer"
actccaggatatttggtcaaaggaaaaggaa

SEQ ID NO: 43 - DNA, 23 bp, Artificial Sequence
  source: /note="Description of Artificial Sequence: Synthetic primer"
agacaccaaaacacctggtcatg

SEQ ID NO: 44 - DNA, 24 bp, Artificial Sequence
  source: /note="Description of Artificial Sequence: Synthetic primer"
agactattcatcaatggccagcga

SEQ ID NO: 45 - DNA, 25 bp, Artificial Sequence
  source: /note="Description of Artificial Sequence: Synthetic primer"
agagcccaagatacaagatcacaga

SEQ ID NO: 46 - DNA, 23 bp, Artificial Sequence
  source: /note="Description of Artificial Sequence: Synthetic primer"
agccacagcgtaatagagaaggg

SEQ ID NO: 47 - DNA, 26 bp, Artificial Sequence
  source: /note="Description of Artificial Sequence: Synthetic primer"
aggacatttggtcaaaggaaaaggac

SEQ ID NO: 48 - DNA, 25 bp, Artificial Sequence
  source: /note="Description of Artificial Sequence: Synthetic primer"
agtccccaagacatctgatcaaaga

SEQ ID NO: 49 - DNA, 23 bp, Artificial Sequence
  source: /note="Description of Artificial Sequence: Synthetic primer"
agtccctgagacacaaggtagca

SEQ ID NO: 50 - DNA, 33 bp, Artificial Sequence
  source: /note="Description of Artificial Sequence: Synthetic primer"
agtctcccagatataagattatagagaaaaggc

SEQ ID NO: 51 - DNA, 23 bp, Artificial Sequence
  source: /note="Description of Artificial Sequence: Synthetic primer"
agtctcccaggtacaaagtcaca

SEQ ID NO: 52 - DNA, 32 bp, Artificial Sequence
  source: /note="Description of Artificial Sequence: Synthetic primer"
agtggttcagtctcccagatataagattatag

SEQ ID NO: 53 - DNA, 24 bp, Artificial Sequence
  source: /note="Description of Artificial Sequence: Synthetic primer"
agtaacaaggtcacagagaaggga

SEQ ID NO: 54 - DNA, 23 bp, Artificial Sequence
  source: /note="Description of Artificial Sequence: Synthetic primer"
caaaattccgggtcctgaagaca

SEQ ID NO: 55 - DNA, 22 bp, Artificial Sequence
  source: /note="Description of Artificial Sequence: Synthetic primer"
caagacacctggtcaggaggag

SEQ ID NO: 56 - DNA, 26 bp, Artificial Sequence
  source: /note="Description of Artificial Sequence: Synthetic primer"
cagactccaaaacatcttgtcagagg

SEQ ID NO: 57 - DNA, 22 bp, Artificial Sequence
  source: /note="Description of Artificial Sequence: Synthetic primer"
cagccatcaggtcacacagatg

SEQ ID NO: 58 - DNA, 24 bp, Artificial Sequence
  source: /note="Description of Artificial Sequence: Synthetic primer"
ccaaggtacaaagtcgcaaagagg

SEQ ID NO: 59 - DNA, 25 bp, Artificial Sequence
  source: /note="Description of Artificial Sequence: Synthetic primer"
cccaaaattccgcatcctgaagata

SEQ ID NO: 60 - DNA, 26 bp, Artificial Sequence
  source: /note="Description of Artificial Sequence: Synthetic primer"
cccagtcccccagatataagattaca

SEQ ID NO: 61 - DNA, 25 bp, Artificial Sequence
  source: /note="Description of Artificial Sequence: Synthetic primer"
ccctaggtacaaagtcgcaaagaga

SEQ ID NO: 62 - DNA, 22 bp, Artificial Sequence
  source: /note="Description of Artificial Sequence: Synthetic primer"
cgccatgaggtgacagagatgg

SEQ ID NO: 63 - DNA, 21 bp, Artificial Sequence
  source: /note="Description of Artificial Sequence: Synthetic primer"
cggcacgaggtgacagagatg

SEQ ID NO: 64 - DNA, 22 bp, Artificial Sequence
  source: /note="Description of Artificial Sequence: Synthetic primer"
gtcacccaggcacaaagtgaca

SEQ ID NO: 65 - DNA, 29 bp, Artificial Sequence
  source: /note="Description of Artificial Sequence: Synthetic primer"
caagatatctgatcaaaacgagaggacag

SEQ ID NO: 66 - DNA, 28 bp, Artificial Sequence
  source: /note="Description of Artificial Sequence: Synthetic primer"
ccaagatatctgatcaaaacgagaggac

SEQ ID NO: 67 - DNA, 28 bp, Artificial Sequence
  source: /note="Description of Artificial Sequence: Synthetic primer"
ctccaagatatctgatcaaaacgagagg

SEQ ID NO: 68 - DNA, 22 bp, Artificial Sequence
  source: /note="Description of Artificial Sequence: Synthetic primer"
gagaggacagcaagtgacactg

SEQ ID NO: 69 - DNA, 30 bp, Artificial Sequence
  source: /note="Description of Artificial Sequence: Synthetic primer"
gagtcactcaaactccaagatatctgatca

SEQ ID NO: 70 - DNA, 23 bp, Artificial Sequence
  source: /note="Description of Artificial Sequence: Synthetic primer"
gctggagtcactcaaactccaag

SEQ ID NO: 71 - DNA, 29 bp, Artificial Sequence
  source: /note="Description of Artificial Sequence: Synthetic primer"
ggagtcactcaaactccaagatatctgat

SEQ ID NO: 72 - DNA, 21 bp, Artificial Sequence
  source: /note="Description of Artificial Sequence: Synthetic primer"
ggctggagtcactcaaactcc

SEQ ID NO: 73 - DNA, 25 bp, Artificial Sequence
  source: /note="Description of Artificial Sequence: Synthetic primer"
catggtcatccagaacccaagatac

SEQ ID NO: 74 - DNA, 22 bp, Artificial Sequence
  source: /note="Description of Artificial Sequence: Synthetic primer"
ccatggtcatccagaacccaag

SEQ ID NO: 75 - DNA, 22 bp, Artificial Sequence
  source: /note="Description of Artificial Sequence: Synthetic primer"
gatgccatggtcatccagaacc

SEQ ID NO: 76 - DNA, 20 bp, Artificial Sequence
  source: /note="Description of Artificial Sequence: Synthetic primer"
ggaaagccagtgaccctgag

SEQ ID NO: 77 - DNA, 22 bp, Artificial Sequence
  source: /note="Description of Artificial Sequence: Synthetic primer"
ggttacccagtttggaaagcca

SEQ ID NO: 78 - DNA, 21 bp, Artificial Sequence
  source: /note="Description of Artificial Sequence: Synthetic primer"
gtttggaaagccagtgaccct

SEQ ID NO: 79 - DNA, 23 bp, Artificial Sequence
  source: /note="Description of Artificial Sequence: Synthetic primer"
gttacccagtttggaaagccagt

SEQ ID NO: 80 - DNA, 20 bp, Artificial Sequence
  source: /note="Description of Artificial Sequence: Synthetic primer"
tgccatggtcatccagaacc

SEQ ID NO: 81 - DNA, 23 bp, Artificial Sequence
  source: /note="Description of Artificial Sequence: Synthetic primer"
ttacccagtttggaaagccagtg

SEQ ID NO: 82 - DNA, 21 bp, Artificial Sequence
  source: /note="Description of Artificial Sequence: Synthetic primer"
tttggaaagccagtgaccctg

SEQ ID NO: 83 - DNA, 28 bp, Artificial Sequence
  source: /note="Description of Artificial Sequence: Synthetic primer"
agagctcgagatatctagtcaaaaggac

SEQ ID NO: 84 - DNA, 27 bp, Artificial Sequence
  source: /note="Description of Artificial Sequence: Synthetic primer"
agctcgagatatctagtcaaaaggacg

SEQ ID NO: 85 - DNA, 26 bp, Artificial Sequence
  source: /note="Description of Artificial Sequence: Synthetic primer"
cgagatatctagtcaaaaggacggga

SEQ ID NO: 86 - DNA, 29 bp, Artificial Sequence
  source: /note="Description of Artificial Sequence: Synthetic primer"
gaaagtaacccagagctcgagatatctag

SEQ ID NO: 87 - DNA, 24 bp, Artificial Sequence
  source: /note="Description of Artificial Sequence: Synthetic primer"
gatgtgaaagtaacccagagctcg

SEQ ID NO: 88 - DNA, 27 bp, Artificial Sequence
  source: /note="Description of Artificial Sequence: Synthetic primer"
gtaacccagagctcgagatatctagtc

SEQ ID NO: 89 - DNA, 23 bp, Artificial Sequence
  source: /note="Description of Artificial Sequence: Synthetic primer"
gtgaaagtaacccagagctcgag

SEQ ID NO: 90 - DNA, 25 bp, Artificial Sequence
  source: /note="Description of Artificial Sequence: Synthetic primer"
  source: /note="Description of Combined DNA/RNA Molecule: Synthetic primer"
aaaauacctggucacacagacggga

SEQ ID NO: 91 - DNA, 25 bp, Artificial Sequence
  source: /note="Description of Artificial Sequence: Synthetic primer"
  source: /note="Description of Combined DNA/RNA Molecule: Synthetic primer"
aagataccgggutacccagttugga

SEQ ID NO: 92 - DNA, 30 bp, Artificial Sequence
  source: /note="Description of Artificial Sequence: Synthetic primer"
  source: /note="Description of Combined DNA/RNA Molecule: Synthetic primer"
actcaaacuccaagacatctgaucaaaacg

SEQ ID NO: 93 - DNA, 25 bp, Artificial Sequence
  source: /note="Description of Artificial Sequence: Synthetic primer"
  source: /note="Description of Combined DNA/RNA Molecule: Synthetic primer"
agaaucccagacacaagatcacaaa

SEQ ID NO: 94 - DNA, 25 bp, Artificial Sequence
  source: /note="Description of Artificial Sequence: Synthetic primer"
  source: /note="Description of Combined DNA/RNA Molecule: Synthetic primer"
agaguccaagacacaagatcacaga

SEQ ID NO: 95 - DNA, 25 bp, Artificial Sequence
  source: /note="Description of Artificial Sequence: Synthetic primer"
  source: /note="Description of Combined DNA/RNA Molecule: Synthetic primer"
agtccccaagacauctgaucagaga

SEQ ID NO: 96 - DNA, 21 bp, Artificial Sequence
  source: /note="Description of Artificial Sequence: Synthetic primer"
  source: /note="Description of Combined DNA/RNA Molecule: Synthetic primer"
atcaauggccagcgacccugg

SEQ ID NO: 97 - DNA, 25 bp, Artificial Sequence
  source: /note="Description of Artificial Sequence: Synthetic primer"
  source: /note="Description of Combined DNA/RNA Molecule: Synthetic primer"
ccaaagucccacacacctgaucaaa

SEQ ID NO: 98 - RNA, 21 nt, Artificial Sequence
  source: /note="Description of Artificial Sequence: Synthetic primer"
cccagacaccaaaauaccugg

SEQ ID NO: 99 - DNA, 27 bp, Artificial Sequence
  source: /note="Description of Artificial Sequence: Synthetic primer"
  source: /note="Description of Combined DNA/RNA Molecule: Synthetic primer"
ctcaacatccgaguagggttatctgua

SEQ ID NO: 100 - DNA, 21 bp, Artificial Sequence
  source: /note="Description of Artificial Sequence: Synthetic primer"
  source: /note="Description of Combined DNA/RNA Molecule: Synthetic primer"
ctcaguccccaaagtaccugt

SEQ ID NO: 101 - RNA, 19 nt, Artificial Sequence
  source: /note="Description of Artificial Sequence: Synthetic primer"
cuggaaucacccagagccc

SEQ ID NO: 102 - DNA, 19 bp, Artificial Sequence
  source: /note="Description of Artificial Sequence: Synthetic primer"
  source: /note="Description of Combined DNA/RNA Molecule: Synthetic primer"
cuggagtcucccacaaccc

SEQ ID NO: 103 - DNA, 19 bp, Artificial Sequence
  source: /note="Description of Artificial Sequence: Synthetic primer"
  source: /note="Description of Combined DNA/RNA Molecule: Synthetic primer"
cuggagtcucccagaaccc

SEQ ID NO: 104 - DNA, 19 bp, Artificial Sequence
  source: /note="Description of Artificial Sequence: Synthetic primer"
  source: /note="Description of Combined DNA/RNA Molecule: Synthetic primer"
cuggagtcucccaggaccc

SEQ ID NO: 105 - DNA, 28 bp, Artificial Sequence
  source: /note="Description of Artificial Sequence: Synthetic primer"
  source: /note="Description of Combined DNA/RNA Molecule: Synthetic primer"
ctggagtcacucaaactccaagatauct

SEQ ID NO: 106 - DNA, 22 bp, Artificial Sequence
  source: /note="Description of Artificial Sequence: Synthetic primer"
  source: /note="Description of Combined DNA/RNA Molecule: Synthetic primer"
gaaagccagugaccctgagtug

SEQ ID NO: 107 - DNA, 25 bp, Artificial Sequence
  source: /note="Description of Artificial Sequence: Synthetic primer"
  source: /note="Description of Combined DNA/RNA Molecule: Synthetic primer"
cccagagcucgagatatctagucaa

SEQ ID NO: 108 - DNA, 24 bp, Artificial Sequence
  source: /note="Description of Artificial Sequence: Synthetic primer"
  source: /note="Description of Combined DNA/RNA Molecule: Synthetic primer"
aaaagccaagcagggauatctguc

SEQ ID NO: 109 - DNA, 25 bp, Artificial Sequence
  source: /note="Description of Artificial Sequence: Synthetic primer"
  source: /note="Description of Combined DNA/RNA Molecule: Synthetic primer"
aaaatacctggucacacagauggga

SEQ ID NO: 110 - DNA, 24 bp, Artificial Sequence
  source: /note="Description of Artificial Sequence: Synthetic primer"
  source: /note="Description of Combined DNA/RNA Molecule: Synthetic primer"
aaaatuccacgtccugaagacagg

SEQ ID NO: 111 - DNA, 24 bp, Artificial Sequence
  source: /note="Description of Artificial Sequence: Synthetic primer"
  source: /note="Description of Combined DNA/RNA Molecule: Synthetic primer"
aaaatuccaggtccugaagacagg

SEQ ID NO: 112 - DNA, 26 bp, Artificial Sequence
  source: /note="Description of Artificial Sequence: Synthetic primer"
  source: /note="Description of Combined DNA/RNA Molecule: Synthetic primer"
aaaautccacatccugaagacaggac

SEQ ID NO: 113 - DNA, 23 bp, Artificial Sequence
  source: /note="Description of Artificial Sequence: Synthetic primer"
  source: /note="Description of Combined DNA/RNA Molecule: Synthetic primer"
aaagcacctgaucacagcaacug

SEQ ID NO: 114 - DNA, 24 bp, Artificial Sequence
  source: /note="Description of Artificial Sequence: Synthetic primer"
  source: /note="Description of Combined DNA/RNA Molecule: Synthetic primer"
aacatccgagcagggutatctgua

SEQ ID NO: 115 - DNA, 24 bp, Artificial Sequence
  source: /note="Description of Artificial Sequence: Synthetic primer"
  source: /note="Description of Combined DNA/RNA Molecule: Synthetic primer"
aacatccgagcugggttatctgua

SEQ ID NO: 116 - DNA, 26 bp, Artificial Sequence
  source: /note="Description of Artificial Sequence: Synthetic primer"
  source: /note="Description of Combined DNA/RNA Molecule: Synthetic primer"
aacccaagauacctcatcacagugac

SEQ ID NO: 117 - DNA, 24 bp, Artificial Sequence
  source: /note="Description of Artificial Sequence: Synthetic primer"
  source: /note="Description of Combined DNA/RNA Molecule: Synthetic primer"
aagacacagaaucatugggacagg

SEQ ID NO: 118 - DNA, 24 bp, Artificial Sequence
  source: /note="Description of Artificial Sequence: Synthetic primer"
  source: /note="Description of Combined DNA/RNA Molecule: Synthetic primer"
aagcatgaggugacagaaauggga

SEQ ID NO: 119 - RNA, 22 nt, Artificial Sequence
  source: /note="Description of Artificial Sequence: Synthetic primer"
aaggcacaaggugacagagaug

SEQ ID NO: 120 - DNA, 24 bp, Artificial Sequence
  source: /note="Description of Artificial Sequence: Synthetic primer"
  source: /note="Description of Combined DNA/RNA Molecule: Synthetic primer"
aatacctggucacacagaugggaa

SEQ ID NO: 121 - DNA, 29 bp, Artificial Sequence
  source: /note="Description of Artificial Sequence: Synthetic primer"
  source: /note="Description of Combined DNA/RNA Molecule: Synthetic primer"
aattcucaagacacagaatcatugggaca

SEQ ID NO: 122 - DNA, 25 bp, Artificial Sequence
  source: /note="Description of Artificial Sequence: Synthetic primer"
  source: /note="Description of Combined DNA/RNA Molecule: Synthetic primer"
acaaagucccacacacctgaucaaa

SEQ ID NO: 123 - RNA, 21 nt, Artificial Sequence
  source: /note="Description of Artificial Sequence: Synthetic primer"
acacaaggucaccaacauggg

SEQ ID NO: 124 - DNA, 21 bp, Artificial Sequence
  source: /note="Description of Artificial Sequence: Synthetic primer"
  source: /note="Description of Combined DNA/RNA Molecule: Synthetic primer"
acaccaagacaccuggtcaug

SEQ ID NO: 125 - DNA, 22 bp, Artificial Sequence
  source: /note="Description of Artificial Sequence: Synthetic primer"
  source: /note="Description of Combined DNA/RNA Molecule: Synthetic primer"
accaacatcucagatccuggca

SEQ ID NO: 126 - DNA, 26 bp, Artificial Sequence
  source: /note="Description of Artificial Sequence: Synthetic primer"
  source: /note="Description of Combined DNA/RNA Molecule: Synthetic primer"
accagaccccaagauaccttgttaua

SEQ ID NO: 127 - RNA, 25 nt, Artificial Sequence
  source: /note="Description of Artificial Sequence: Synthetic primer"
accccaaggaauaggaucacaaaga

SEQ ID NO: 128 - RNA, 21 nt, Artificial Sequence
  source: /note="Description of Artificial Sequence: Synthetic primer"
acccccaguaacaaggucaca

SEQ ID NO: 129 - DNA, 26 bp, Artificial Sequence
  source: /note="Description of Artificial Sequence: Synthetic primer"
  source: /note="Description of Combined DNA/RNA Molecule: Synthetic primer"
acctagacttcuggtcaaagcaagug

SEQ ID NO: 130 - DNA, 27 bp, Artificial Sequence
  source: /note="Description of Artificial Sequence: Synthetic primer"
  source: /note="Description of Combined DNA/RNA Molecule: Synthetic primer"
acctagatttcuggtcaaagcaaauga

SEQ ID NO: 131 - DNA, 31 bp, Artificial Sequence
  source: /note="Description of Artificial Sequence: Synthetic primer"
  source: /note="Description of Combined DNA/RNA Molecule: Synthetic primer"
acuccaggatatttggucaaaggaaaaggaa

SEQ ID NO: 132 - DNA, 23 bp, Artificial Sequence
  source: /note="Description of Artificial Sequence: Synthetic primer"
  source: /note="Description of Combined DNA/RNA Molecule: Synthetic primer"
agacaccaaaacaccuggtcaug

SEQ ID NO: 133 - DNA, 24 bp, Artificial Sequence
  source: /note="Description of Artificial Sequence: Synthetic primer"
  source: /note="Description of Combined DNA/RNA Molecule: Synthetic primer"
agacuattcatcaauggccagcga

SEQ ID NO: 134 - RNA, 25 nt, Artificial Sequence
  source: /note="Description of Artificial Sequence: Synthetic primer"
agagcccaagauacaagaucacaga

SEQ ID NO: 135 - RNA, 23 nt, Artificial Sequence
  source: /note="Description of Artificial Sequence: Synthetic primer"
agccacagcguaauagagaaggg

SEQ ID NO: 136 - DNA, 26 bp, Artificial Sequence
  source: /note="Description of Artificial Sequence: Synthetic primer"
  source: /note="Description of Combined DNA/RNA Molecule: Synthetic primer"
aggacauttggucaaaggaaaaggac

SEQ ID NO: 137 - DNA, 25 bp, Artificial Sequence
  source: /note="Description of Artificial Sequence: Synthetic primer"
  source: /note="Description of Combined DNA/RNA Molecule: Synthetic primer"
agtccccaagacauctgaucaaaga

SEQ ID NO: 138 - DNA, 23 bp, Artificial Sequence
  source: /note="Description of Artificial Sequence: Synthetic primer"
  source: /note="Description of Combined DNA/RNA Molecule: Synthetic primer"
agtcccugagacacaagguagca

SEQ ID NO: 139 - DNA, 33 bp, Artificial Sequence
  source: /note="Description of Artificial Sequence: Synthetic primer"
  source: /note="Description of Combined DNA/RNA Molecule: Synthetic primer"
agtctcccagauataagattauagagaaaaggc

SEQ ID NO: 140 - DNA, 23 bp, Artificial Sequence
  source: /note="Description of Artificial Sequence: Synthetic primer"
  source: /note="Description of Combined DNA/RNA Molecule: Synthetic primer"
agtctcccagguacaaagucaca

SEQ ID NO: 141 - DNA, 32 bp, Artificial Sequence
  source: /note="Description of Artificial Sequence: Synthetic primer"
  source: /note="Description of Combined DNA/RNA Molecule: Synthetic primer"
agtggttcagtcucccagatataagattauag

SEQ ID NO: 142 - RNA, 24 nt, Artificial Sequence
  source: /note="Description of Artificial Sequence: Synthetic primer"
aguaacaaggucacagagaaggga

SEQ ID NO: 143 - DNA, 23 bp, Artificial Sequence
  source: /note="Description of Artificial Sequence: Synthetic primer"
  source: /note="Description of Combined DNA/RNA Molecule: Synthetic primer"
caaaatuccgggtccugaagaca

SEQ ID NO: 144 - RNA, 22 nt, Artificial Sequence
  source: /note="Description of Artificial Sequence: Synthetic primer"
caagacaccuggucaggaggag

SEQ ID NO: 145 - DNA, 26 bp, Artificial Sequence
  source: /note="Description of Artificial Sequence: Synthetic primer"
  source: /note="Description of Combined DNA/RNA Molecule: Synthetic primer"
cagacuccaaaacatcttgucagagg

SEQ ID NO: 146 - DNA, 22 bp, Artificial Sequence
  source: /note="Description of Artificial Sequence: Synthetic primer"
  source: /note="Description of Combined DNA/RNA Molecule: Synthetic primer"
cagccatcaggucacacagaug

SEQ ID NO: 147 - RNA, 24 nt, Artificial Sequence
  source: /note="Description of Artificial Sequence: Synthetic primer"
ccaagguacaaagucgcaaagagg

SEQ ID NO: 148 - DNA, 25 bp, Artificial Sequence
  source: /note="Description of Artificial Sequence: Synthetic primer"
  source: /note="Description of Combined DNA/RNA Molecule: Synthetic primer"
cccaaaattccgcaucctgaagaua

SEQ ID NO: 149 - DNA, 26 bp, Artificial Sequence
  source: /note="Description of Artificial Sequence: Synthetic primer"
  source: /note="Description of Combined DNA/RNA Molecule: Synthetic primer"
cccagucccccagatataagatuaca

SEQ ID NO: 150 - DNA, 25 bp, Artificial Sequence
  source: /note="Description of Artificial Sequence: Synthetic primer"
  source: /note="Description of Combined DNA/RNA Molecule: Synthetic primer"
cccuaggtacaaagucgcaaagaga

SEQ ID NO: 151 - DNA, 22 bp, Artificial Sequence
  source: /note="Description of Artificial Sequence: Synthetic primer"
  source: /note="Description of Combined DNA/RNA Molecule: Synthetic primer"
cgccatgaggugacagagaugg

SEQ ID NO: 152 - RNA, 21 nt, Artificial Sequence
  source: /note="Description of Artificial Sequence: Synthetic primer"
cggcacgaggugacagagaug

SEQ ID NO: 153 - RNA, 22 nt, Artificial Sequence
  source: /note="Description of Artificial Sequence: Synthetic primer"
gucacccaggcacaaagugaca

SEQ ID NO: 154 - RNA, 25 nt, Artificial Sequence
  source: /note="Description of Artificial Sequence: Synthetic primer"
agaguccaagacacaagaucacaga

SEQ ID NO: 155 - RNA, 25 nt, Artificial Sequence
  source: /note="Description of Artificial Sequence: Synthetic primer"
agaaucccagacacaagaucacaaa

SEQ ID NO: 156 - DNA, 28 bp, Artificial Sequence
  source: /note="Description of Artificial Sequence: Synthetic primer"
  source: /note="Description of Combined DNA/RNA Molecule: Synthetic primer"
cuccaagatatctgaucaaaacgagagg

SEQ ID NO: 157 - RNA, 22 nt, Artificial Sequence
  source: /note="Description of Artificial Sequence: Synthetic primer"
gagaggacagcaagugacacug

SEQ ID NO: 158 - DNA, 30 bp, Artificial Sequence
  source: /note="Description of Artificial Sequence: Synthetic primer"
  source: /note="Description of Combined DNA/RNA Molecule: Synthetic primer"
gagtcactcaaacuccaagatatctgauca

SEQ ID NO: 159 - DNA, 23 bp, Artificial Sequence
  source: /note="Description of Artificial Sequence: Synthetic primer"
  source: /note="Description of Combined DNA/RNA Molecule: Synthetic primer"
gctggagucactcaaacuccaag

SEQ ID NO: 160 - DNA, 29 bp, Artificial Sequence
  source: /note="Description of Artificial Sequence: Synthetic primer"
  source: /note="Description of Combined DNA/RNA Molecule: Synthetic primer"
ggagtcactcaaacuccaagatatcugat

SEQ ID NO: 161 - DNA, 21 bp, Artificial Sequence
  source: /note="Description of Artificial Sequence: Synthetic primer"
  source: /note="Description of Combined DNA/RNA Molecule: Synthetic primer"
ggctggagucactcaaacucc

SEQ ID NO: 162 - DNA, 25 bp, Artificial Sequence
  source: /note="Description of Artificial Sequence: Synthetic primer"
  source: /note="Description of Combined DNA/RNA Molecule: Synthetic primer"
catggtcauccagaacccaagauac

SEQ ID NO: 163 - DNA, 22 bp, Artificial Sequence
  source: /note="Description of Artificial Sequence: Synthetic primer"
  source: /note="Description of Combined DNA/RNA Molecule: Synthetic primer"
ccauggtcauccagaacccaag

SEQ ID NO: 164 - DNA, 22 bp, Artificial Sequence
  source: /note="Description of Artificial Sequence: Synthetic primer"
  source: /note="Description of Combined DNA/RNA Molecule: Synthetic primer"
gatgccauggtcauccagaacc

SEQ ID NO: 165 - RNA, 20 nt, Artificial Sequence
  source: /note="Description of Artificial Sequence: Synthetic primer"
ggaaagccagugacccugag

SEQ ID NO: 166 - DNA, 22 bp, Artificial Sequence
  source: /note="Description of Artificial Sequence: Synthetic primer"
  source: /note="Description of Combined DNA/RNA Molecule: Synthetic primer"
ggutacccagttuggaaagcca

SEQ ID NO: 167 - DNA, 21 bp, Artificial Sequence
  source: /note="Description of Artificial Sequence: Synthetic primer"
  source: /note="Description of Combined DNA/RNA Molecule: Synthetic primer"
gttuggaaagccagugaccct

SEQ ID NO: 168 - DNA, 23 bp, Artificial Sequence
  source: /note="Description of Artificial Sequence: Synthetic primer"
  source: /note="Description of Combined DNA/RNA Molecule: Synthetic primer"
gutacccagttuggaaagccagt

SEQ ID NO: 169 - DNA, 20 bp, Artificial Sequence
  source: /note="Description of Artificial Sequence: Synthetic primer"
  source: /note="Description of Combined DNA/RNA Molecule: Synthetic primer"
tgccauggtcauccagaacc

SEQ ID NO: 170 - DNA, 23 bp, Artificial Sequence
  source: /note="Description of Artificial Sequence: Synthetic primer"
  source: /note="Description of Combined DNA/RNA Molecule: Synthetic primer"
ttacccagttuggaaagccagug

SEQ ID NO: 171 - DNA, 21 bp, Artificial Sequence
  source: /note="Description of Artificial Sequence: Synthetic primer"
  source: /note="Description of Combined DNA/RNA Molecule: Synthetic primer"
tttggaaagccagugacccug

SEQ ID NO: 172 - DNA, 28 bp, Artificial Sequence
  source: /note="Description of Artificial Sequence: Synthetic primer"
  source: /note="Description of Combined DNA/RNA Molecule: Synthetic primer"
agagcucgagatatctagucaaaaggac

SEQ ID NO: 173 - DNA, 27 bp, Artificial Sequence
  source: /note="Description of Artificial Sequence: Synthetic primer"
  source: /note="Description of Combined DNA/RNA Molecule: Synthetic primer"
agctcgagauatctagucaaaaggacg

SEQ ID NO: 174 - DNA, 26 bp, Artificial Sequence
  source: /note="Description of Artificial Sequence: Synthetic primer"
  source: /note="Description of Combined DNA/RNA Molecule: Synthetic primer"
cgagauatctagucaaaaggacggga

SEQ ID NO: 175 - DNA, 29 bp, Artificial Sequence
  source: /note="Description of Artificial Sequence: Synthetic primer"
  source: /note="Description of Combined DNA/RNA Molecule: Synthetic primer"
gaaagtaacccagagcucgagatatcuag

SEQ ID NO: 176 - DNA, 24 bp, Artificial Sequence
  source: /note="Description of Artificial Sequence: Synthetic primer"
  source: /note="Description of Combined DNA/RNA Molecule: Synthetic primer"
gatgtgaaaguaacccagagcucg

SEQ ID NO: 177 - DNA, 27 bp, Artificial Sequence
  source: /note="Description of Artificial Sequence: Synthetic primer"
  source: /note="Description of Combined DNA/RNA Molecule: Synthetic primer"
gtaacccagagcucgagatatctaguc

SEQ ID NO: 178 - DNA, 23 bp, Artificial Sequence
  source: /note="Description of Artificial Sequence: Synthetic primer"
  source: /note="Description of Combined DNA/RNA Molecule: Synthetic primer"
gtgaaaguaacccagagcucgag

SEQ ID NO: 179 - DNA, 29 bp, Artificial Sequence
  source: /note="Description of Artificial Sequence: Synthetic primer"
  source: /note="Description of Combined DNA/RNA Molecule: Synthetic primer"
caagauatctgaucaaaacgagaggacag

SEQ ID NO: 180 - DNA, 28 bp, Artificial Sequence
  source: /note="Description of Artificial Sequence: Synthetic primer"
  source: /note="Description of Combined DNA/RNA Molecule: Synthetic primer"
ccaagauatctgaucaaaacgagaggac

SEQ ID NO: 181 - DNA, 7 bp, Artificial Sequence
  source: /note="Description of Artificial Sequence: Synthetic oligonucleotide"
aattggt

SEQ ID NO: 182 - DNA, 7 bp, Artificial Sequence
  source: /note="Description of Artificial Sequence: Synthetic oligonucleotide"
aaatggt

SEQ ID NO: 183 - DNA, 10 bp, Artificial Sequence
  source: /note="Description of Artificial Sequence: Synthetic oligonucleotide"
aaaatttggt

SEQ ID NO: 184 - DNA, 22 bp, Artificial Sequence
  source: /note="Description of Artificial Sequence: Synthetic oligonucleotide"
aaaatttttatccccccccggg

SEQ ID NO: 185 - DNA, 24 bp, Artificial Sequence
  source: /note="Description of Artificial Sequence: Synthetic primer"
aatcttcacatcaattccctggag

SEQ ID NO: 186 - DNA, 17 bp, Artificial Sequence
  source: /note="Description of Artificial Sequence: Synthetic primer"
acatccgctcaccaggc

SEQ ID NO: 187 - DNA, 18 bp, Artificial Sequence
  source: /note="Description of Artificial Sequence: Synthetic primer"
acctacacaccctgcagc

SEQ ID NO: 188 - DNA, 17 bp, Artificial Sequence
  source: /note="Description of Artificial Sequence: Synthetic primer"
aggctggagtcagctgc

SEQ ID NO: 189 - DNA, 17 bp, Artificial Sequence
  source: /note="Description of Artificial Sequence: Synthetic primer"
aggtgcagcctgcagaa

SEQ ID NO: 190 - DNA, 21 bp, Artificial Sequence
  source: /note="Description of Artificial Sequence: Synthetic primer"
atgaatgtgagcaccttggag

SEQ ID NO: 191 - DNA, 21 bp, Artificial Sequence
  source: /note="Description of Artificial Sequence: Synthetic primer"
atgaatgtgagtgccttggag

SEQ ID NO: 192 - DNA, 18 bp, Artificial Sequence
  source: /note="Description of Artificial Sequence: Synthetic primer"
caagctggagtcagctgc

SEQ ID NO: 193 - DNA, 19 bp, Artificial Sequence
  source: /note="Description of Artificial Sequence: Synthetic primer"
catgagctccttggagctg

SEQ ID NO: 194 - DNA, 25 bp, Artificial Sequence
  source: /note="Description of Artificial Sequence: Synthetic primer"
cattctgagttctaagaagctcctc

SEQ ID NO: 195 - DNA, 19 bp, Artificial Sequence
  source: /note="Description of Artificial Sequence: Synthetic primer"
cctgaccctgaagtctgct

SEQ ID NO: 196 - DNA, 19 bp, Artificial Sequence
  source: /note="Description of Artificial Sequence: Synthetic primer"
cctgagctctctggagctg

SEQ ID NO: 197 - DNA, 21 bp, Artificial Sequence
  source: /note="Description of Artificial Sequence: Synthetic primer"
ctagacatccgctcaccaggc

SEQ ID NO: 198 - DNA, 21 bp, Artificial Sequence
  source: /note="Description of Artificial Sequence: Synthetic primer"
ctcaagatccagcctgcaaag

SEQ ID NO: 199 - DNA, 21 bp, Artificial Sequence
  source: /note="Description of Artificial Sequence: Synthetic primer"
ctcaagatccagcctgcagag

SEQ ID NO: 200 - DNA, 21 bp, Artificial Sequence
  source: /note="Description of Artificial Sequence: Synthetic primer"
ctcacgttggcgtctgctgta

SEQ ID NO: 201 - DNA, 21 bp, Artificial Sequence
  source: /note="Description of Artificial Sequence: Synthetic primer"
ctcactctggagtcagctacc

SEQ ID NO: 202 - DNA, 21 bp, Artificial Sequence
  source: /note="Description of Artificial Sequence: Synthetic primer"
ctcactctggagtccgctacc

SEQ ID NO: 203 - DNA, 21 bp, Artificial Sequence
  source: /note="Description of Artificial Sequence: Synthetic primer"
ctcactctggagtctgctgcc

SEQ ID NO: 204 - DNA, 21 bp, Artificial Sequence
  source: /note="Description of Artificial Sequence: Synthetic primer"
ctcactgtgacatcggcccaa

SEQ ID NO: 205 - DNA, 21 bp, Artificial Sequence
  source: /note="Description of Artificial Sequence: Synthetic primer"
ctgaagatccagccctcagaa

SEQ ID NO: 206 - DNA, 21 bp, Artificial Sequence
  source: /note="Description of Artificial Sequence: Synthetic primer"
ctgaagatccagcctgcagag

SEQ ID NO: 207 - DNA, 21 bp, Artificial Sequence
  source: /note="Description of Artificial Sequence: Synthetic primer"
ctgaagatccggtccacaaag

SEQ ID NO: 208 - DNA, 21 bp, Artificial Sequence
  source: /note="Description of Artificial Sequence: Synthetic primer"
ctgaatgtgaacgccttgttg

SEQ ID NO: 209 - DNA, 21 bp, Artificial Sequence
  source: /note="Description of Artificial Sequence: Synthetic primer"
ctgaatgtgaacgccttggag

SEQ ID NO: 210 - DNA, 21 bp, Artificial Sequence
  source: /note="Description of Artificial Sequence: Synthetic primer"
ctgacagtgaccagtgcccat

SEQ ID NO: 211 - DNA, 21 bp, Artificial Sequence
  source: /note="Description of Artificial Sequence: Synthetic primer"
ctgacagtgacctgtgcccat

SEQ ID NO: 212 - DNA, 21 bp, Artificial Sequence
  source: /note="Description of Artificial Sequence: Synthetic primer"
ctgaccctgaagtctgccagc

SEQ ID NO: 213 - DNA, 21 bp, Artificial Sequence
  source: /note="Description of Artificial Sequence: Synthetic primer"
ctgactgtgagcaacatgagc

SEQ ID NO: 214 - DNA, 21 bp, Artificial Sequence
  source: /note="Description of Artificial Sequence: Synthetic primer"
ctgaggatccagcaggtagtg

SEQ ID NO: 215 - DNA, 21 bp, Artificial Sequence
  source: /note="Description of Artificial Sequence: Synthetic primer"
ctgaggatccagcccatggaa

SEQ ID NO: 216 - DNA, 21 bp, Artificial Sequence
  source: /note="Description of Artificial Sequence: Synthetic primer"
ctgaggatccagccctcagaa

SEQ ID NO: 217 - DNA, 21 bp, Artificial Sequence
  source: /note="Description of Artificial Sequence: Synthetic primer"
ctggcaatcctgtcctcagaa

SEQ ID NO: 218 - DNA, 21 bp, Artificial Sequence
  source: /note="Description of Artificial Sequence: Synthetic primer"
ctggcaatcctgtcctcggaa

SEQ ID NO: 219 - DNA, 21 bp, Artificial Sequence
  source: /note="Description of Artificial Sequence: Synthetic primer"
ctgtccctagagtctgccatc

SEQ ID NO: 220 - DNA, 21 bp, Artificial Sequence
  source: /note="Description of Artificial Sequence: Synthetic primer"
ctcaagatccagccagcagag

SEQ ID NO: 221 - DNA, 21 bp, Artificial Sequence
  source: /note="Description of Artificial Sequence: Synthetic primer"
ctgaagatccatcccgcagag

SEQ ID NO: 222 - DNA, 21 bp, Artificial Sequence
  source: /note="Description of Artificial Sequence: Synthetic primer"
ctgaagatccagcgcacacag

SEQ ID NO: 223 - DNA, 21 bp, Artificial Sequence
  source: /note="Description of Artificial Sequence: Synthetic primer"
ctgaagatccagcgcacagag

SEQ ID NO: 224 - DNA, 21 bp, Artificial Sequence
  source: /note="Description of Artificial Sequence: Synthetic primer"
ctgaagttccagcgcacacag

SEQ ID NO: 225 - DNA, 21 bp, Artificial Sequence
  source: /note="Description of Artificial Sequence: Synthetic primer"
ctgacgattcagcgcacagag

SEQ ID NO: 226 - DNA, 18 bp, Artificial Sequence
  source: /note="Description of Artificial Sequence: Synthetic primer"
ctgacgatccagcgcaca

SEQ ID NO: 227 - DNA, 21 bp, Artificial Sequence
  source: /note="Description of Artificial Sequence: Synthetic primer"
ctgactgtgagcaacaggaga

SEQ ID NO: 228 - DNA, 21 bp, Artificial Sequence
  source: /note="Description of Artificial Sequence: Synthetic primer"
ctgattctggagtccgccagc

SEQ ID NO: 229 - DNA, 20 bp, Artificial Sequence
  source: /note="Description of Artificial Sequence: Synthetic primer"
gccttgagatccaggctacg

SEQ ID NO: 230 - DNA, 17 bp, Artificial Sequence
  source: /note="Description of Artificial Sequence: Synthetic primer"
ggctggagttggctgct

SEQ ID NO: 231 - DNA, 17 bp, Artificial Sequence
  source: /note="Description of Artificial Sequence: Synthetic primer"
ggttggagtcggctgct

SEQ ID NO: 232 - DNA, 17 bp, Artificial Sequence
  source: /note="Description of Artificial Sequence: Synthetic primer"
tcacctacacgccctgc

SEQ ID NO: 233 - DNA, 17 bp, Artificial Sequence
  source: /note="Description of Artificial Sequence: Synthetic primer"
tcaggctgctgtcggct

SEQ ID NO: 234 - DNA, 17 bp, Artificial Sequence
  source: /note="Description of Artificial Sequence: Synthetic primer"
tcaggctggagtcggct

SEQ ID NO: 235 - DNA, 17 bp, Artificial Sequence
  source: /note="Description of Artificial Sequence: Synthetic primer"
tcaggctggtgtcggct

SEQ ID NO: 236 - DNA, 24 bp, Artificial Sequence
  source: /note="Description of Artificial Sequence: Synthetic primer"
tcatcctgagttctaagaagctcc

SEQ ID NO: 237 - DNA, 23 bp, Artificial Sequence
  source: /note="Description of Artificial Sequence: Synthetic primer"
tcctgagttctaagaagctcctc

SEQ ID NO: 238 - DNA, 22 bp, Artificial Sequence
  source: /note="Description of Artificial Sequence: Synthetic primer"
tctcaagatccaacctgcaaag

SEQ ID NO: 239 - DNA, 17 bp, Artificial Sequence
  source: /note="Description of Artificial Sequence: Synthetic primer"
tgaccctggagtctgcc

SEQ ID NO: 240 - DNA, 17 bp, Artificial Sequence
  source: /note="Description of Artificial Sequence: Synthetic primer"
tgatcctggagtcgccc

SEQ ID NO: 241 - DNA, 17 bp, Artificial Sequence
  source: /note="Description of Artificial Sequence: Synthetic primer"
tgtggtcgcactgcagc

SEQ ID NO: 242 - DNA, 21 bp, Artificial Sequence
  source: /note="Description of Artificial Sequence: Synthetic primer"
ttggagatccagtccacggag

SEQ ID NO: 243 - DNA, 21 bp, Artificial Sequence
  source: /note="Description of Artificial Sequence: Synthetic primer"
ttggagatccagcgcacagag

SEQ ID NO: 244 - DNA, 20 bp, Artificial Sequence
  source: /note="Description of Artificial Sequence: Synthetic primer"
catgagctccttggagctgg

SEQ ID NO: 245 - DNA, 21 bp, Artificial Sequence
  source: /note="Description of Artificial Sequence: Synthetic primer"
aacatgagctccttggagctg

SEQ ID NO: 246 - DNA, 22 bp, Artificial Sequence
  source: /note="Description of Artificial Sequence: Synthetic primer"
gaacatgagctccttggagctg

SEQ ID NO: 247 - DNA, 23 bp, Artificial Sequence
  source: /note="Description of Artificial Sequence: Synthetic primer"
tgaactgaacatgagctccttgg

SEQ ID NO: 248 - DNA, 24 bp, Artificial Sequence
  source: /note="Description of Artificial Sequence: Synthetic primer"
ctgaactgaacatgagctccttgg

SEQ ID NO: 249 - DNA, 24 bp, Artificial Sequence
  source: /note="Description of Artificial Sequence: Synthetic primer"
  source: /note="Description of Combined DNA/RNA Molecule: Synthetic primer"
aatcttcacaucaattcccuggag

SEQ ID NO: 250 - RNA, 17 nt, Artificial Sequence
  source: /note="Description of Artificial Sequence: Synthetic primer"
acauccgcucaccaggc

SEQ ID NO: 251 - RNA, 18 nt, Artificial Sequence
  source: /note="Description of Artificial Sequence: Synthetic primer"
accuacacacccugcagc

SEQ ID NO: 252 - DNA, 17 bp, Artificial Sequence
  source: /note="Description of Artificial Sequence: Synthetic primer"
  source: /note="Description of Combined DNA/RNA Molecule: Synthetic primer"
aggcuggagtcagcugc

SEQ ID NO: 253 - RNA, 17 nt, Artificial Sequence
  source: /note="Description of Artificial Sequence: Synthetic primer"
aggugcagccugcagaa

SEQ ID NO: 254 - DNA, 21 bp, Artificial Sequence
  source: /note="Description of Artificial Sequence: Synthetic primer"
  source: /note="Description of Combined DNA/RNA Molecule: Synthetic primer"
atgaatgugagcacctuggag

SEQ ID NO: 255 - DNA, 21 bp, Artificial Sequence
  source: /note="Description of Artificial Sequence: Synthetic primer"
  source: /note="Description of Combined DNA/RNA Molecule: Synthetic primer"
atgaatgugagtgcctuggag

SEQ ID NO: 256 - DNA, 18 bp, Artificial Sequence
  source: /note="Description of Artificial Sequence: Synthetic primer"
  source: /note="Description of Combined DNA/RNA Molecule: Synthetic primer"
caagcuggagtcagcugc

SEQ ID NO: 257 - DNA, 19 bp, Artificial Sequence
  source: /note="Description of Artificial Sequence: Synthetic primer"
  source: /note="Description of Combined DNA/RNA Molecule: Synthetic primer"
catgagcuccttggagcug

SEQ ID NO: 258 - DNA, 25 bp, Artificial Sequence
  source: /note="Description of Artificial Sequence: Synthetic primer"
  source: /note="Description of Combined DNA/RNA Molecule: Synthetic primer"
cattctgagttcuaagaagctccuc

SEQ ID NO: 259 - DNA, 19 bp, Artificial Sequence
  source: /note="Description of Artificial Sequence: Synthetic primer"
  source: /note="Description of Combined DNA/RNA Molecule: Synthetic primer"
cctgacccugaagtcugct

SEQ ID NO: 260 - DNA, 19 bp, Artificial Sequence
  source: /note="Description of Artificial Sequence: Synthetic primer"
  source: /note="Description of Combined DNA/RNA Molecule: Synthetic primer"
cctgagcuctctggagcug

SEQ ID NO: 261 - DNA, 21 bp, Artificial Sequence
  source: /note="Description of Artificial Sequence: Synthetic primer"
  source: /note="Description of Combined DNA/RNA Molecule: Synthetic primer"
ctagacauccgcucaccaggc

SEQ ID NO: 262 - DNA, 21 bp, Artificial Sequence
  source: /note="Description of Artificial Sequence: Synthetic primer"
  source: /note="Description of Combined DNA/RNA Molecule: Synthetic primer"
ctcaagauccagccugcaaag

SEQ ID NO: 263 - DNA, 21 bp, Artificial Sequence
  source: /note="Description of Artificial Sequence: Synthetic primer"
  source: /note="Description of Combined DNA/RNA Molecule: Synthetic primer"
ctcaagauccagccugcagag

SEQ ID NO: 264 - DNA, 21 bp, Artificial Sequence
  source: /note="Description of Artificial Sequence: Synthetic primer"
  source: /note="Description of Combined DNA/RNA Molecule: Synthetic primer"
ctcacgtuggcgtctgctgua

SEQ ID NO: 265 - DNA, 21 bp, Artificial Sequence
  source: /note="Description of Artificial Sequence: Synthetic primer"
  source: /note="Description of Combined DNA/RNA Molecule: Synthetic primer"
ctcactcuggagtcagcuacc

SEQ ID NO: 266 - DNA, 21 bp, Artificial Sequence
  source: /note="Description of Artificial Sequence: Synthetic primer"
  source: /note="Description of Combined DNA/RNA Molecule: Synthetic primer"
ctcactcuggagtccgcuacc

SEQ ID NO: 267 - DNA, 21 bp, Artificial Sequence
  source: /note="Description of Artificial Sequence: Synthetic primer"
  source: /note="Description of Combined DNA/RNA Molecule: Synthetic primer"
ctcactcuggagtctgcugcc

SEQ ID NO: 268 - DNA, 21 bp, Artificial Sequence
  source: /note="Description of Artificial Sequence: Synthetic primer"
  source: /note="Description of Combined DNA/RNA Molecule: Synthetic primer"
ctcacugtgacaucggcccaa

SEQ ID NO: 269 - DNA, 21 bp, Artificial Sequence
  source: /note="Description of Artificial Sequence: Synthetic primer"
  source: /note="Description of Combined DNA/RNA Molecule: Synthetic primer"
ctgaagauccagcccucagaa

SEQ ID NO: 270 - DNA, 21 bp, Artificial Sequence
  source: /note="Description of Artificial Sequence: Synthetic primer"
  source: /note="Description of Combined DNA/RNA Molecule: Synthetic primer"
ctgaagauccagccugcagag

SEQ ID NO: 271 - DNA, 21 bp, Artificial Sequence
  source: /note="Description of Artificial Sequence: Synthetic primer"
  source: /note="Description of Combined DNA/RNA Molecule: Synthetic primer"
ctgaagauccgguccacaaag

SEQ ID NO: 272 - DNA, 21 bp, Artificial Sequence
  source: /note="Description of Artificial Sequence: Synthetic primer"
  source: /note="Description of Combined DNA/RNA Molecule: Synthetic primer"
ctgaatgugaacgccttgtug

SEQ ID NO: 273 - DNA, 21 bp, Artificial Sequence
  source: /note="Description of Artificial Sequence: Synthetic primer"
  source: /note="Description of Combined DNA/RNA Molecule: Synthetic primer"
ctgaatgugaacgcctuggag

SEQ ID NO: 274 - DNA, 21 bp, Artificial Sequence
  source: /note="Description of Artificial Sequence: Synthetic primer"
  source: /note="Description of Combined DNA/RNA Molecule: Synthetic primer"
ctgacagugaccagugcccat

SEQ ID NO: 275 - DNA, 21 bp, Artificial Sequence
  source: /note="Description of Artificial Sequence: Synthetic primer"
  source: /note="Description of Combined DNA/RNA Molecule: Synthetic primer"
ctgacagugacctgugcccat

SEQ ID NO: 276 - DNA, 21 bp, Artificial Sequence
  source: /note="Description of Artificial Sequence: Synthetic primer"
  source: /note="Description of Combined DNA/RNA Molecule: Synthetic primer"
ctgacccugaagtcugccagc

SEQ ID NO: 277 - DNA, 21 bp, Artificial Sequence
  source: /note="Description of Artificial Sequence: Synthetic primer"
  source: /note="Description of Combined DNA/RNA Molecule: Synthetic primer"
ctgactgugagcaacaugagc

SEQ ID NO: 278 - DNA, 21 bp, Artificial Sequence
  source: /note="Description of Artificial Sequence: Synthetic primer"
  source: /note="Description of Combined DNA/RNA Molecule: Synthetic primer"
ctgaggauccagcaggtagug

SEQ ID NO: 279 - DNA, 21 bp, Artificial Sequence
  source: /note="Description of Artificial Sequence: Synthetic primer"
  source: /note="Description of Combined DNA/RNA Molecule: Synthetic primer"
ctgaggauccagcccauggaa

SEQ ID NO: 280 - DNA, 21 bp, Artificial Sequence
  source: /note="Description of Artificial Sequence: Synthetic primer"
  source: /note="Description of Combined DNA/RNA Molecule: Synthetic primer"
ctgaggauccagcccucagaa

SEQ ID NO: 281 - DNA, 21 bp, Artificial Sequence
  source: /note="Description of Artificial Sequence: Synthetic primer"
  source: /note="Description of Combined DNA/RNA Molecule: Synthetic primer"
ctggcaaucctgtccucagaa

SEQ ID NO: 282 - DNA, 21 bp, Artificial Sequence
  source: /note="Description of Artificial Sequence: Synthetic primer"
  source: /note="Description of Combined DNA/RNA Molecule: Synthetic primer"
ctggcaaucctgtccucggaa

SEQ ID NO: 283 - DNA, 21 bp, Artificial Sequence
  source: /note="Description of Artificial Sequence: Synthetic primer"
  source: /note="Description of Combined DNA/RNA Molecule: Synthetic primer"
ctgtcccuagagtctgccauc

SEQ ID NO: 284 - RNA, 21 nt, Artificial Sequence
  source: /note="Description of Artificial Sequence: Synthetic primer"
cucaagauccagccagcagag

SEQ ID NO: 285 - DNA, 21 bp, Artificial Sequence
  source: /note="Description of Artificial Sequence: Synthetic primer"
  source: /note="Description of Combined DNA/RNA Molecule: Synthetic primer"
cugaagatccaucccgcagag

SEQ ID NO: 286 - RNA, 21 nt, Artificial Sequence
  source: /note="Description of Artificial Sequence: Synthetic primer"
cugaagauccagcgcacacag

SEQ ID NO: 287 - RNA, 21 nt, Artificial Sequence
  source: /note="Description of Artificial Sequence: Synthetic primer"
cugaagauccagcgcacagag

SEQ ID NO: 288 - DNA, 21 bp, Artificial Sequence
  source: /note="Description of Artificial Sequence: Synthetic primer"
  source: /note="Description of Combined DNA/RNA Molecule: Synthetic primer"
cugaagtuccagcgcacacag

SEQ ID NO: 289 - DNA, 21 bp, Artificial Sequence
  source: /note="Description of Artificial Sequence: Synthetic primer"
  source: /note="Description of Combined DNA/RNA Molecule: Synthetic primer"
cugacgatucagcgcacagag

SEQ ID NO: 290 - RNA, 18 nt, Artificial Sequence
  source: /note="Description of Artificial Sequence: Synthetic primer"
cugacgauccagcgcaca

SEQ ID NO: 291 - DNA, 21 bp, Artificial Sequence
  source: /note="Description of Artificial Sequence: Synthetic primer"
  source: /note="Description of Combined DNA/RNA Molecule: Synthetic primer"
cugactgugagcaacaggaga

SEQ ID NO: 292 - DNA, 21 bp, Artificial Sequence
  source: /note="Description of Artificial Sequence: Synthetic primer"
  source: /note="Description of Combined DNA/RNA Molecule: Synthetic primer"
cugattctggaguccgccagc

SEQ ID NO: 293 - DNA, 20 bp, Artificial Sequence
  source: /note="Description of Artificial Sequence: Synthetic primer"
  source: /note="Description of Combined DNA/RNA Molecule: Synthetic primer"
gccttgagauccaggcuacg

SEQ ID NO: 294 - DNA, 17 bp, Artificial Sequence
  source: /note="Description of Artificial Sequence: Synthetic primer"
  source: /note="Description of Combined DNA/RNA Molecule: Synthetic primer"
ggctggagutggcugct

SEQ ID NO: 295 - DNA, 17 bp, Artificial Sequence
  source: /note="Description of Artificial Sequence: Synthetic primer"
  source: /note="Description of Combined DNA/RNA Molecule: Synthetic primer"
ggttggagucggcugct

SEQ ID NO: 296 - DNA, 17 bp, Artificial Sequence
  source: /note="Description of Artificial Sequence: Synthetic primer"
  source: /note="Description of Combined DNA/RNA Molecule: Synthetic primer"
tcaccuacacgcccugc

SEQ ID NO: 297 - DNA, 17 bp, Artificial Sequence
  source: /note="Description of Artificial Sequence: Synthetic primer"
  source: /note="Description of Combined DNA/RNA Molecule: Synthetic primer"
tcaggcugctgucggct

SEQ ID NO: 298 - DNA, 17 bp, Artificial Sequence
  source: /note="Description of Artificial Sequence: Synthetic primer"
  source: /note="Description of Combined DNA/RNA Molecule: Synthetic primer"
tcaggcuggagucggct

SEQ ID NO: 299 - DNA, 17 bp, Artificial Sequence
  source: /note="Description of Artificial Sequence: Synthetic primer"
  source: /note="Description of Combined DNA/RNA Molecule: Synthetic primer"
tcaggcuggtgucggct

SEQ ID NO: 300 - DNA, 24 bp, Artificial Sequence
  source: /note="Description of Artificial Sequence: Synthetic primer"
  source: /note="Description of Combined DNA/RNA Molecule: Synthetic primer"
tcatcctgagutctaagaagcucc

SEQ ID NO: 301 - DNA, 23 bp, Artificial Sequence
  source: /note="Description of Artificial Sequence: Synthetic primer"
  source: /note="Description of Combined DNA/RNA Molecule: Synthetic primer"
tcctgagttcuaagaagctccuc

SEQ ID NO: 302 - DNA, 22 bp, Artificial Sequence
  source: /note="Description of Artificial Sequence: Synthetic primer"
  source: /note="Description of Combined DNA/RNA Molecule: Synthetic primer"
tctcaagauccaaccugcaaag

SEQ ID NO: 303 - DNA, 17 bp, Artificial Sequence
  source: /note="Description of Artificial Sequence: Synthetic primer"
  source: /note="Description of Combined DNA/RNA Molecule: Synthetic primer"
tgacccuggagtcugcc

SEQ ID NO: 304 - DNA, 17 bp, Artificial Sequence
  source: /note="Description of Artificial Sequence: Synthetic primer"
  source: /note="Description of Combined DNA/RNA Molecule: Synthetic primer"
tgatccuggagucgccc

SEQ ID NO: 305 - DNA, 17 bp, Artificial Sequence
  source: /note="Description of Artificial Sequence: Synthetic primer"
  source: /note="Description of Combined DNA/RNA Molecule: Synthetic primer"
tgtggucgcacugcagc

SEQ ID NO: 306 - DNA, 21 bp, Artificial Sequence
  source: /note="Description of Artificial Sequence: Synthetic primer"
  source: /note="Description of Combined DNA/RNA Molecule: Synthetic primer"
ttggagauccaguccacggag

SEQ ID NO: 307 - DNA, 21 bp, Artificial Sequence
  source: /note="Description of Artificial Sequence: Synthetic primer"
  source: /note="Description of Combined DNA/RNA Molecule: Synthetic primer"
tuggagauccagcgcacagag

SEQ ID NO: 308 - DNA, 20 bp, Artificial Sequence
  source: /note="Description of Artificial Sequence: Synthetic primer"
  source: /note="Description of Combined DNA/RNA Molecule: Synthetic primer"
catgagcuccttggagcugg

SEQ ID NO: 309 - DNA, 21 bp, Artificial Sequence
  source: /note="Description of Artificial Sequence: Synthetic primer"
  source: /note="Description of Combined DNA/RNA Molecule: Synthetic primer"
aacatgagcuccttggagcug

SEQ ID NO: 310 - DNA, 22 bp, Artificial Sequence
  source: /note="Description of Artificial Sequence: Synthetic primer"
  source: /note="Description of Combined DNA/RNA Molecule: Synthetic primer"
gaacatgagcuccttggagcug

SEQ ID NO: 311 - DNA, 23 bp, Artificial Sequence
  source: /note="Description of Artificial Sequence: Synthetic primer"
  source: /note="Description of Combined DNA/RNA Molecule: Synthetic primer"
tgaactgaacaugagctcctugg

SEQ ID NO: 312 - DNA, 24 bp, Artificial Sequence
  source: /note="Description of Artificial Sequence: Synthetic primer"
  source: /note="Description of Combined DNA/RNA Molecule: Synthetic primer"
ctgaactgaacaugagctcctugg

SEQ ID NO: 313 - DNA, 17 bp, Artificial Sequence
  source: /note="Description of Artificial Sequence: Synthetic primer"
aaccaggagtcctccgc

SEQ ID NO: 314 - DNA, 19 bp, Artificial Sequence
  source: /note="Description of Artificial Sequence: Synthetic primer"
acggtcagcctagagcctt

SEQ ID NO: 315 - DNA, 19 bp, Artificial Sequence
  source: /note="Description of Artificial Sequence: Synthetic primer"
agtctggtgccttgtccaa

SEQ ID NO: 316 - DNA, 17 bp, Artificial Sequence
  source: /note="Description of Artificial Sequence: Synthetic primer"
cacggtcagcctgctgc

SEQ ID NO: 317 - DNA, 20 bp, Artificial Sequence
  source: /note="Description of Artificial Sequence: Synthetic primer"
cccatcaccaaaatgctggg

SEQ ID NO: 318 - DNA, 19 bp, Artificial Sequence
  source: /note="Description of Artificial Sequence: Synthetic primer"
cctgggccaaaatactgcg

SEQ ID NO: 319 - DNA, 17 bp, Artificial Sequence
  source: /note="Description of Artificial Sequence: Synthetic primer"
cggcccgaagtactgct

SEQ ID NO: 320 - DNA, 17 bp, Artificial Sequence
  source: /note="Description of Artificial Sequence: Synthetic primer"
cggcgccgaagtactga

SEQ ID NO: 321 - DNA, 17 bp, Artificial Sequence
  source: /note="Description of Artificial Sequence: Synthetic primer"
ctggcccgaagaactgc

SEQ ID NO: 322 - DNA, 20 bp, Artificial Sequence
  source: /note="Description of Artificial Sequence: Synthetic primer"
gagccaacttccctctccaa

SEQ ID NO: 323 - DNA, 19 bp, Artificial Sequence
  source: /note="Description of Artificial Sequence: Synthetic primer"
gcctggtcccattcccaaa

SEQ ID NO: 324 - DNA, 19 bp, Artificial Sequence
  source: /note="Description of Artificial Sequence: Synthetic primer"
gctgggttccactgccaaa

SEQ ID NO: 325 - DNA, 19 bp, Artificial Sequence
  source: /note="Description of Artificial Sequence: Synthetic primer"
tcccgttcccaaagtggag

SEQ ID NO: 326 - DNA, 17 bp, Artificial Sequence
  source: /note="Description of Artificial Sequence: Synthetic primer"
tgaccgtgagcctggtg

SEQ ID NO: 327 - DNA, 17 bp, Artificial Sequence
  source: /note="Description of Artificial Sequence: Synthetic primer"
tggcccgaagtactggg

SEQ ID NO: 328 - DNA, 19 bp, Artificial Sequence
  source: /note="Description of Artificial Sequence: Synthetic primer"
ttaacctggtccccgaacc

SEQ ID NO: 329 - DNA, 17 bp, Artificial Sequence
  source: /note="Description of Artificial Sequence: Synthetic primer"
gaccgtgagcctggtgc

SEQ ID NO: 330 - DNA, 17 bp, Artificial Sequence
  source: /note="Description of Artificial Sequence: Synthetic primer"
caggagccgcgtgcctg

SEQ ID NO: 331 - DNA, 17 bp, Artificial Sequence
  source: /note="Description of Artificial Sequence: Synthetic primer"
agcactgtcagccgggt

SEQ ID NO: 332 - DNA, 17 bp, Artificial Sequence
  source: /note="Description of Artificial Sequence: Synthetic primer"
ccagcacggtcagcctg

SEQ ID NO: 333 - DNA, 17 bp, Artificial Sequence
  source: /note="Description of Artificial Sequence: Synthetic primer"
ctagcacggtgagccgt

SEQ ID NO: 334 - DNA, 18 bp, Artificial Sequence
  source: /note="Description of Artificial Sequence: Synthetic primer"
agcactgagagccgggtc

SEQ ID NO: 335 - DNA, 20 bp, Artificial Sequence
  source: /note="Description of Artificial Sequence: Synthetic primer"
cagtacggtcagcctagagc

SEQ ID NO: 336 - DNA, 20 bp, Artificial Sequence
  source: /note="Description of Artificial Sequence: Synthetic primer"
ccagaaccaggagtcctccg

SEQ ID NO: 337 - DNA, 20 bp, Artificial Sequence
  source: /note="Description of Artificial Sequence: Synthetic primer"
ctgtcacagtgagcctggtc

SEQ ID NO: 338 - DNA, 21 bp, Artificial Sequence
  source: /note="Description of Artificial Sequence: Synthetic primer"
ccaagacagagagctgggttc

SEQ ID NO: 339 - DNA, 22 bp, Artificial Sequence
  source: /note="Description of Artificial Sequence: Synthetic primer"
ctacaactgtgagtctggtgcc

SEQ ID NO: 340 - DNA, 22 bp, Artificial Sequence
  source: /note="Description of Artificial Sequence: Synthetic primer"
ctaggatggagagtcgagtccc

SEQ ID NO: 341 - DNA, 22 bp, Artificial Sequence
  source: /note="Description of Artificial Sequence: Synthetic primer"
ctacaacggttaacctggtccc

SEQ ID NO: 342 - DNA, 23 bp, Artificial Sequence
  source: /note="Description of Artificial Sequence: Synthetic primer"
ctacaacagtgagccaacttccc

SEQ ID NO: 343 - DNA, 17 bp, Artificial Sequence
  source: /note="Description of Artificial Sequence: Synthetic primer"
gtgaccgtgagcctggt

SEQ ID NO: 344 - DNA, 17 bp, Artificial Sequence
  source: /note="Description of Artificial Sequence: Synthetic primer"
tgtgaccgtgagcctgg

SEQ ID NO: 345 - DNA, 18 bp, Artificial Sequence
  source: /note="Description of Artificial Sequence: Synthetic primer"
gtgaccgtgagcctggtg

SEQ ID NO: 346 - DNA, 18 bp, Artificial Sequence
  source: /note="Description of Artificial Sequence: Synthetic primer"
tgtgaccgtgagcctggt

SEQ ID NO: 347 - DNA, 18 bp, Artificial Sequence
  source: /note="Description of Artificial Sequence: Synthetic primer"
ctgtgaccgtgagcctgg

SEQ ID NO: 348 - DNA, 17 bp, Artificial Sequence
  source: /note="Description of Artificial Sequence: Synthetic primer"
caggagtcctccgccca

SEQ ID NO: 349 - DNA, 17 bp, Artificial Sequence
  source: /note="Description of Artificial Sequence: Synthetic primer"
accaggagtcctccgcc

SEQ ID NO: 350 - DNA, 17 bp, Artificial Sequence
  source: /note="Description of Artificial Sequence: Synthetic primer"
actgagagccgggtccc

SEQ ID NO: 351 - DNA, 17 bp, Artificial Sequence
  source: /note="Description of Artificial Sequence: Synthetic primer"
cactgagagccgggtcc

SEQ ID NO: 352 - DNA, 17 bp, Artificial Sequence
  source: /note="Description of Artificial Sequence: Synthetic primer"
gcactgagagccgggtc

SEQ ID NO: 353 - DNA, 17 bp, Artificial Sequence
  source: /note="Description of Artificial Sequence: Synthetic primer"
gcacggtcagcctgctg

SEQ ID NO: 354 - DNA, 17 bp, Artificial Sequence
  source: /note="Description of Artificial Sequence: Synthetic primer"
cagcacggtcagcctgc

SEQ ID NO: 355 - DNA, 17 bp, Artificial Sequence
  source: /note="Description of Artificial Sequence: Synthetic primer"
tagcacggtgagccgtg

SEQ ID NO: 356 - DNA, 18 bp, Artificial Sequence
  source: /note="Description of Artificial Sequence: Synthetic primer"
ccaggagccgcgtgcctg

SEQ ID NO: 357 - DNA, 18 bp, Artificial Sequence
  source: /note="Description of Artificial Sequence: Synthetic primer"
aaccaggagtcctccgcc

SEQ ID NO: 358 - DNA, 18 bp, Artificial Sequence
  source: /note="Description of Artificial Sequence: Synthetic primer"
gaaccaggagtcctccgc

SEQ ID NO: 359 - DNA, 18 bp, Artificial Sequence
  source: /note="Description of Artificial Sequence: Synthetic primer"
tagcacggtgagccgtgt

SEQ ID NO: 360 - DNA, 19 bp, Artificial Sequence
  source: /note="Description of Artificial Sequence: Synthetic primer"
accaggagccgcgtgcctg

SEQ ID NO: 361 - DNA, 19 bp, Artificial Sequence
  source: /note="Description of Artificial Sequence: Synthetic primer"
aacggttaacctggtcccc

SEQ ID NO: 362 - DNA, 19 bp, Artificial Sequence
  source: /note="Description of Artificial Sequence: Synthetic primer"
agaaccaggagtcctccgc

SEQ ID NO: 363 - DNA, 19 bp, Artificial Sequence
  source: /note="Description of Artificial Sequence: Synthetic primer"
cagaaccaggagtcctccg

SEQ ID NO: 364 - DNA, 20 bp, Artificial Sequence
  source: /note="Description of Artificial Sequence: Synthetic primer"
tacggtcagcctagagcctt

SEQ ID NO: 365 - DNA, 20 bp, Artificial Sequence
  source: /note="Description of Artificial Sequence: Synthetic primer"
gtacggtcagcctagagcct

SEQ ID NO: 366 - DNA, 20 bp, Artificial Sequence
  source: /note="Description of Artificial Sequence: Synthetic primer"
ggatggagagtcgagtccca

SEQ ID NO: 367 - DNA, 20 bp, Artificial Sequence
  source: /note="Description of Artificial Sequence: Synthetic primer"
caacggttaacctggtcccc

SEQ ID NO: 368 - DNA, 20 bp, Artificial Sequence
  source: /note="Description of Artificial Sequence: Synthetic primer"
agtacggtcagcctagagcc

SEQ ID NO: 369 - DNA, 20 bp, Artificial Sequence
  source: /note="Description of Artificial Sequence: Synthetic primer"
aggatggagagtcgagtccc

SEQ ID NO: 370 - DNA, 20 bp, Artificial Sequence
  source: /note="Description of Artificial Sequence: Synthetic primer"
acaacggttaacctggtccc

SEQ ID NO: 371 - DNA, 20 bp, Artificial Sequence
  source: /note="Description of Artificial Sequence: Synthetic primer"
tgtcacagtgagcctggtcc

SEQ ID NO: 372 - DNA, 21 bp, Artificial Sequence
  source: /note="Description of Artificial Sequence: Synthetic primer"
caactgtgagtctggtgcctt

SEQ ID NO: 373 - DNA, 21 bp, Artificial Sequence
  source: /note="Description of Artificial Sequence: Synthetic primer"
gtacggtcagcctagagcctt

SEQ ID NO: 374 - DNA, 21 bp, Artificial Sequence
  source: /note="Description of Artificial Sequence: Synthetic primer"
ggatggagagtcgagtcccat

SEQ ID NO: 375 - DNA, 21 bp, Artificial Sequence
  source: /note="Description of Artificial Sequence: Synthetic primer"
acaactgtgagtctggtgcct

SEQ ID NO: 376 - DNA, 21 bp, Artificial Sequence
  source: /note="Description of Artificial Sequence: Synthetic primer"
agtacggtcagcctagagcct

SEQ ID NO: 377 - DNA, 21 bp, Artificial Sequence
  source: /note="Description of Artificial Sequence: Synthetic primer"
aggatggagagtcgagtccca

SEQ ID NO: 378 - DNA, 21 bp, Artificial Sequence
  source: /note="Description of Artificial Sequence: Synthetic primer"
tacaactgtgagtctggtgcc

SEQ ID NO: 379 - DNA, 21 bp, Artificial Sequence
  source: /note="Description of Artificial Sequence: Synthetic primer"
caagacagagagctgggttcc

SEQ ID NO: 380 - DNA, 21 bp, Artificial Sequence
  source: /note="Description of Artificial Sequence: Synthetic primer"
taggatggagagtcgagtccc

SEQ ID NO: 381 - DNA, 21 bp, Artificial Sequence
  source: /note="Description of Artificial Sequence: Synthetic primer"
tacaacggttaacctggtccc

SEQ ID NO: 382 - DNA, 22 bp, Artificial Sequence
  source: /note="Description of Artificial Sequence: Synthetic primer"
acaactgtgagtctggtgcctt

SEQ ID NO: 383 - DNA, 22 bp, Artificial Sequence
  source: /note="Description of Artificial Sequence: Synthetic primer"
aagacagagagctgggttccac

SEQ ID NO: 384 - DNA, 22 bp, Artificial Sequence
  source: /note="Description of Artificial Sequence: Synthetic primer"
aggatggagagtcgagtcccat

SEQ ID NO: 385 - DNA, 22 bp, Artificial Sequence
  source: /note="Description of Artificial Sequence: Synthetic primer"
acaacagtgagccaacttccct

SEQ ID NO: 386 - DNA, 22 bp, Artificial Sequence
  source: /note="Description of Artificial Sequence: Synthetic primer"
tacaactgtgagtctggtgcct

SEQ ID NO: 387 - DNA, 22 bp, Artificial Sequence
  source: /note="Description of Artificial Sequence: Synthetic primer"
caagacagagagctgggttcca

SEQ ID NO: 388 - DNA, 22 bp, Artificial Sequence
  source: /note="Description of Artificial Sequence: Synthetic primer"
taggatggagagtcgagtccca

SEQ ID NO: 389 - DNA, 22 bp, Artificial Sequence
  source: /note="Description of Artificial Sequence: Synthetic primer"
tacaacggttaacctggtcccc

SEQ ID NO: 390 - DNA, 23 bp, Artificial Sequence
  source: /note="Description of Artificial Sequence: Synthetic primer"
tacaactgtgagtctggtgcctt

SEQ ID NO: 391 - DNA, 23 bp, Artificial Sequence
  source: /note="Description of Artificial Sequence: Synthetic primer"
taggatggagagtcgagtcccat

SEQ ID NO: 392 - DNA, 23 bp, Artificial Sequence
  source: /note="Description of Artificial Sequence: Synthetic primer"
tacaacagtgagccaacttccct

SEQ ID NO: 393 - DNA, 23 bp, Artificial Sequence
  source: /note="Description of Artificial Sequence: Synthetic primer"
ctacaactgtgagtctggtgcct

SEQ ID NO: 394 - DNA, 23 bp, Artificial Sequence
  source: /note="Description of Artificial Sequence: Synthetic primer"
ctaggatggagagtcgagtccca

SEQ ID NO: 395 - DNA, 24 bp, Artificial Sequence
  source: /note="Description of Artificial Sequence: Synthetic primer"
ctacaactgtgagtctggtgcctt

SEQ ID NO: 396 - DNA, 24 bp, Artificial Sequence
  source: /note="Description of Artificial Sequence: Synthetic primer"
ctaggatggagagtcgagtcccat

SEQ ID NO: 397 - DNA, 24 bp, Artificial Sequence
  source: /note="Description of Artificial Sequence: Synthetic primer"
ctacaacagtgagccaacttccct

SEQ ID NO: 398 - RNA, 17 nt, Artificial Sequence
  source: /note="Description of Artificial Sequence: Synthetic primer"
aaccaggaguccuccgc

SEQ ID NO: 399 - DNA, 19 bp, Artificial Sequence
  source: /note="Description of Artificial Sequence: Synthetic primer"
  source: /note="Description of Combined DNA/RNA Molecule: Synthetic primer"
acggtcagccuagagccut

SEQ ID NO: 400 - DNA, 19 bp, Artificial Sequence
  source: /note="Description of Artificial Sequence: Synthetic primer"
  source: /note="Description of Combined DNA/RNA Molecule: Synthetic primer"
agtctggugccttguccaa

SEQ ID NO: 401 - DNA, 17 bp, Artificial Sequence
  source: /note="Description of Artificial Sequence: Synthetic primer"
  source: /note="Description of Combined DNA/RNA Molecule: Synthetic primer"
cacggucagcctgcugc

SEQ ID NO: 402 - DNA, 20 bp, Artificial Sequence
  source: /note="Description of Artificial Sequence: Synthetic primer"
  source: /note="Description of Combined DNA/RNA Molecule: Synthetic primer"
cccaucaccaaaatgcuggg

SEQ ID NO: 403 - DNA, 19 bp, Artificial Sequence
  source: /note="Description of Artificial Sequence: Synthetic primer"
  source: /note="Description of Combined DNA/RNA Molecule: Synthetic primer"
ccugggccaaaatacugcg

SEQ ID NO: 404 - DNA, 17 bp, Artificial Sequence
  source: /note="Description of Artificial Sequence: Synthetic primer"
  source: /note="Description of Combined DNA/RNA Molecule: Synthetic primer"
cggcccgaaguacugct

SEQ ID NO: 405 - RNA, 17 nt, Artificial Sequence
  source: /note="Description of Artificial Sequence: Synthetic primer"
cggcgccgaaguacuga

SEQ ID NO: 406 - RNA, 17 nt, Artificial Sequence
  source: /note="Description of Artificial Sequence: Synthetic primer"
cuggcccgaagaacugc

SEQ ID NO: 407 - DNA, 20 bp, Artificial Sequence
  source: /note="Description of Artificial Sequence: Synthetic primer"
  source: /note="Description of Combined DNA/RNA Molecule: Synthetic primer"
gagccaacutccctcuccaa

SEQ ID NO: 408 - DNA, 19 bp, Artificial Sequence
  source: /note="Description of Artificial Sequence: Synthetic primer"
  source: /note="Description of Combined DNA/RNA Molecule: Synthetic primer"
gcctggucccatucccaaa

SEQ ID NO: 409 - DNA, 19 bp, Artificial Sequence
  source: /note="Description of Artificial Sequence: Synthetic primer"
  source: /note="Description of Combined DNA/RNA Molecule: Synthetic primer"
gctgggutccacugccaaa

SEQ ID NO: 410 - DNA, 19 bp, Artificial Sequence
  source: /note="Description of Artificial Sequence: Synthetic primer"
  source: /note="Description of Combined DNA/RNA Molecule: Synthetic primer"
tcccgtucccaaaguggag

SEQ ID NO: 411 - DNA, 17 bp, Artificial Sequence
  source: /note="Description of Artificial Sequence: Synthetic primer"
  source: /note="Description of Combined DNA/RNA Molecule: Synthetic primer"
tgaccgugagcctggug

SEQ ID NO: 412 - DNA, 17 bp, Artificial Sequence
  source: /note="Description of Artificial Sequence: Synthetic primer"
  source: /note="Description of Combined DNA/RNA Molecule: Synthetic primer"
tggcccgaaguacuggg

SEQ ID NO: 413 - DNA, 19 bp, Artificial Sequence
  source: /note="Description of Artificial Sequence: Synthetic primer"
  source: /note="Description of Combined DNA/RNA Molecule: Synthetic primer"
tuaacctgguccccgaacc

SEQ ID NO: 414 - DNA, 17 bp, Artificial Sequence
  source: /note="Description of Artificial Sequence: Synthetic primer"
  source: /note="Description of Combined DNA/RNA Molecule: Synthetic primer"
gaccgugagcctggugc

SEQ ID NO: 415 - RNA, 17 nt, Artificial Sequence
  source: /note="Description of Artificial Sequence: Synthetic primer"
caggagccgcgugccug

SEQ ID NO: 416 - DNA, 17 bp, Artificial Sequence
  source: /note="Description of Artificial Sequence: Synthetic primer"
  source: /note="Description of Combined DNA/RNA Molecule: Synthetic primer"
agcacugucagccgggt

SEQ ID NO: 417 - RNA, 17 nt, Artificial Sequence
  source: /note="Description of Artificial Sequence: Synthetic primer"
ccagcacggucagccug

SEQ ID NO: 418 - DNA, 17 bp, Artificial Sequence
  source: /note="Description of Artificial Sequence: Synthetic primer"
  source: /note="Description of Combined DNA/RNA Molecule: Synthetic primer"
cuagcacggugagccgt

SEQ ID NO: 419 - RNA, 18 nt, Artificial Sequence
  source: /note="Description of Artificial Sequence: Synthetic primer"
agcacugagagccggguc

SEQ ID NO: 420 - DNA, 20 bp, Artificial Sequence
  source: /note="Description of Artificial Sequence: Synthetic primer"
  source: /note="Description of Combined DNA/RNA Molecule: Synthetic primer"
cagtacggucagccuagagc

SEQ ID NO: 421 - RNA, 20 nt, Artificial Sequence
  source: /note="Description of Artificial Sequence: Synthetic primer"
ccagaaccaggaguccuccg

SEQ ID NO: 422 - DNA, 20 bp, Artificial Sequence
  source: /note="Description of Artificial Sequence: Synthetic primer"
  source: /note="Description of Combined DNA/RNA Molecule: Synthetic primer"
ctgtcacagugagcctgguc

SEQ ID NO: 423 - DNA, 21 bp, Artificial Sequence
  source: /note="Description of Artificial Sequence: Synthetic primer"
  source: /note="Description of Combined DNA/RNA Molecule: Synthetic primer"
ccaagacagagagcugggtuc

SEQ ID NO: 424 - DNA, 22 bp, Artificial Sequence
  source: /note="Description of Artificial Sequence: Synthetic primer"
  source: /note="Description of Combined DNA/RNA Molecule: Synthetic primer"
ctacaactgugagtctggugcc

SEQ ID NO: 425 - DNA, 22 bp, Artificial Sequence
  source: /note="Description of Artificial Sequence: Synthetic primer"
  source: /note="Description of Combined DNA/RNA Molecule: Synthetic primer"
ctaggauggagagtcgaguccc

SEQ ID NO: 426 - DNA, 22 bp, Artificial Sequence
  source: /note="Description of Artificial Sequence: Synthetic primer"
  source: /note="Description of Combined DNA/RNA Molecule: Synthetic primer"
ctacaacggutaacctgguccc

SEQ ID NO: 427 - DNA, 23 bp, Artificial Sequence
  source: /note="Description of Artificial Sequence: Synthetic primer"
  source: /note="Description of Combined DNA/RNA Molecule: Synthetic primer"
ctacaacagugagccaactuccc

SEQ ID NO: 428 - DNA, 17 bp, Artificial Sequence
  source: /note="Description of Artificial Sequence: Synthetic primer"
  source: /note="Description of Combined DNA/RNA Molecule: Synthetic primer"
gtgaccgugagccuggt

SEQ ID NO: 429 - DNA, 17 bp, Artificial Sequence
  source: /note="Description of Artificial Sequence: Synthetic primer"
  source: /note="Description of Combined DNA/RNA Molecule: Synthetic primer"
tgtgaccgugagccugg

SEQ ID NO: 430 - DNA, 18 bp, Artificial Sequence
  source: /note="Description of Artificial Sequence: Synthetic primer"
  source: /note="Description of Combined DNA/RNA Molecule: Synthetic primer"
gtgaccgugagcctggug

SEQ ID NO: 431 - DNA, 18 bp, Artificial Sequence
  source: /note="Description of Artificial Sequence: Synthetic primer"
  source: /note="Description of Combined DNA/RNA Molecule: Synthetic primer"
tgtgaccgugagccuggt

SEQ ID NO: 432 - DNA, 18 bp, Artificial Sequence
  source: /note="Description of Artificial Sequence: Synthetic primer"
  source: /note="Description of Combined DNA/RNA Molecule: Synthetic primer"
ctgtgaccgugagccugg

SEQ ID NO: 433 - RNA, 17 nt, Artificial Sequence
  source: /note="Description of Artificial Sequence: Synthetic primer"
caggaguccuccgccca

SEQ ID NO: 434 - RNA, 17 nt, Artificial Sequence
  source: /note="Description of Artificial Sequence: Synthetic primer"
accaggaguccuccgcc

SEQ ID NO: 435 - RNA, 17 nt, Artificial Sequence
  source: /note="Description of Artificial Sequence: Synthetic primer"
acugagagccggguccc

SEQ ID NO: 436 - RNA, 17 nt, Artificial Sequence
  source: /note="Description of Artificial Sequence: Synthetic primer"
cacugagagccgggucc

SEQ ID NO: 437 - RNA, 17 nt, Artificial Sequence
  source: /note="Description of Artificial Sequence: Synthetic primer"
gcacugagagccggguc

SEQ ID NO: 438 - DNA, 17 bp, Artificial Sequence
  source: /note="Description of Artificial Sequence: Synthetic primer"
  source: /note="Description of Combined DNA/RNA Molecule: Synthetic primer"
gcacggucagcctgcug

SEQ ID NO: 439 - RNA, 17 nt, Artificial Sequence
  source: /note="Description of Artificial Sequence: Synthetic primer"
cagcacggucagccugc

SEQ ID NO: 440 - DNA, 17 bp, Artificial Sequence
  source: /note="Description of Artificial Sequence: Synthetic primer"
  source: /note="Description of Combined DNA/RNA Molecule: Synthetic primer"
tagcacggugagccgug

SEQ ID NO: 441 - RNA, 18 nt, Artificial Sequence
  source: /note="Description of Artificial Sequence: Synthetic primer"
ccaggagccgcgugccug

SEQ ID NO: 442 - RNA, 18 nt, Artificial Sequence
  source: /note="Description of Artificial Sequence: Synthetic primer"
aaccaggaguccuccgcc

SEQ ID NO: 443 - RNA, 18 nt, Artificial Sequence
  source: /note="Description of Artificial Sequence: Synthetic primer"
gaaccaggaguccuccgc

SEQ ID NO: 444 - DNA, 18 bp, Artificial Sequence
  source: /note="Description of Artificial Sequence: Synthetic primer"
  source: /note="Description of Combined DNA/RNA Molecule: Synthetic primer"
tagcacggugagccgugt

SEQ ID NO: 445 - RNA, 19 nt, Artificial Sequence
  source: /note="Description of Artificial Sequence: Synthetic primer"
accaggagccgcgugccug

SEQ ID NO: 446 - DNA, 19 bp, Artificial Sequence
  source: /note="Description of Artificial Sequence: Synthetic primer"
  source: /note="Description of Combined DNA/RNA Molecule: Synthetic primer"
aacggtuaacctggucccc

SEQ ID NO: 447 - RNA, 19 nt, Artificial Sequence
  source: /note="Description of Artificial Sequence: Synthetic primer"
agaaccaggaguccuccgc

SEQ ID NO: 448 - RNA, 19 nt, Artificial Sequence
  source: /note="Description of Artificial Sequence: Synthetic primer"
cagaaccaggaguccuccg

SEQ ID NO: 449 - DNA, 20 bp, Artificial Sequence
  source: /note="Description of Artificial Sequence: Synthetic primer"
  source: /note="Description of Combined DNA/RNA Molecule: Synthetic primer"
tacggtcagccuagagccut

SEQ ID NO: 450 - DNA, 20 bp, Artificial Sequence
  source: /note="Description of Artificial Sequence: Synthetic primer"
  source: /note="Description of Combined DNA/RNA Molecule: Synthetic primer"
gtacggucagccuagagcct

SEQ ID NO: 451 - DNA, 20 bp, Artificial Sequence
  source: /note="Description of Artificial Sequence: Synthetic primer"
  source: /note="Description of Combined DNA/RNA Molecule: Synthetic primer"
ggatggagagucgaguccca

SEQ ID NO: 452 - DNA, 20 bp, Artificial Sequence
  source: /note="Description of Artificial Sequence: Synthetic primer"
  source: /note="Description of Combined DNA/RNA Molecule: Synthetic primer"
caacggtuaacctggucccc

SEQ ID NO: 453 - DNA, 20 bp, Artificial Sequence
  source: /note="Description of Artificial Sequence: Synthetic primer"
  source: /note="Description of Combined DNA/RNA Molecule: Synthetic primer"
agtacggucagccuagagcc

SEQ ID NO: 454 - DNA, 20 bp, Artificial Sequence
  source: /note="Description of Artificial Sequence: Synthetic primer"
  source: /note="Description of Combined DNA/RNA Molecule: Synthetic primer"
aggatggagagucgaguccc

SEQ ID NO: 455 - DNA, 20 bp, Artificial Sequence
  source: /note="Description of Artificial Sequence: Synthetic primer"
  source: /note="Description of Combined DNA/RNA Molecule: Synthetic primer"
acaacggutaacctgguccc

SEQ ID NO: 456 - DNA, 20 bp, Artificial Sequence
  source: /note="Description of Artificial Sequence: Synthetic primer"
  source: /note="Description of Combined DNA/RNA Molecule: Synthetic primer"
tgtcacagugagcctggucc

SEQ ID NO: 457 - DNA, 21 bp, Artificial Sequence
  source: /note="Description of Artificial Sequence: Synthetic primer"
  source: /note="Description of Combined DNA/RNA Molecule: Synthetic primer"
caactgtgaguctggtgccut

SEQ ID NO: 458 - DNA, 21 bp, Artificial Sequence
  source: /note="Description of Artificial Sequence: Synthetic primer"
  source: /note="Description of Combined DNA/RNA Molecule: Synthetic primer"
gtacggucagcctagagccut

SEQ ID NO: 459 - DNA, 21 bp, Artificial Sequence
  source: /note="Description of Artificial Sequence: Synthetic primer"
  source: /note="Description of Combined DNA/RNA Molecule: Synthetic primer"
ggatggagagucgagucccat

SEQ ID NO: 460 - DNA, 21 bp, Artificial Sequence
  source: /note="Description of Artificial Sequence: Synthetic primer"
  source: /note="Description of Combined DNA/RNA Molecule: Synthetic primer"
acaactgugagtctggugcct

SEQ ID NO: 461 - DNA, 21 bp, Artificial Sequence
  source: /note="Description of Artificial Sequence: Synthetic primer"
  source: /note="Description of Combined DNA/RNA Molecule: Synthetic primer"
agtacggucagccuagagcct

SEQ ID NO: 462 - DNA, 21 bp, Artificial Sequence
  source: /note="Description of Artificial Sequence: Synthetic primer"
  source: /note="Description of Combined DNA/RNA Molecule: Synthetic primer"
aggatggagagucgaguccca

SEQ ID NO: 463 - DNA, 21 bp, Artificial Sequence
  source: /note="Description of Artificial Sequence: Synthetic primer"
  source: /note="Description of Combined DNA/RNA Molecule: Synthetic primer"
tacaactgugagtctggugcc

SEQ ID NO: 464 - DNA, 21 bp, Artificial Sequence
  source: /note="Description of Artificial Sequence: Synthetic primer"
  source: /note="Description of Combined DNA/RNA Molecule: Synthetic primer"
caagacagagagcugggtucc

SEQ ID NO: 465 - DNA, 21 bp, Artificial Sequence
  source: /note="Description of Artificial Sequence: Synthetic primer"
  source: /note="Description of Combined DNA/RNA Molecule: Synthetic primer"
taggauggagagtcgaguccc

SEQ ID NO: 466 - DNA, 21 bp, Artificial Sequence
  source: /note="Description of Artificial Sequence: Synthetic primer"
  source: /note="Description of Combined DNA/RNA Molecule: Synthetic primer"
tacaacggutaacctgguccc

SEQ ID NO: 467 - DNA, 22 bp, Artificial Sequence
  source: /note="Description of Artificial Sequence: Synthetic primer"
  source: /note="Description of Combined DNA/RNA Molecule: Synthetic primer"
acaactgtgaguctggtgccut

SEQ ID NO: 468 - DNA, 22 bp, Artificial Sequence
  source: /note="Description of Artificial Sequence: Synthetic primer"
  source: /note="Description of Combined DNA/RNA Molecule: Synthetic primer"
aagacagagagcugggtuccac

SEQ ID NO: 469 - DNA, 22 bp, Artificial Sequence
  source: /note="Description of Artificial Sequence: Synthetic primer"
  source: /note="Description of Combined DNA/RNA Molecule: Synthetic primer"
aggatggagagucgagucccat

SEQ ID NO: 470 - DNA, 22 bp, Artificial Sequence
  source: /note="Description of Artificial Sequence: Synthetic primer"
  source: /note="Description of Combined DNA/RNA Molecule: Synthetic primer"
acaacagugagccaactuccct

SEQ ID NO: 471 - DNA, 22 bp, Artificial Sequence
  source: /note="Description of Artificial Sequence: Synthetic primer"
  source: /note="Description of Combined DNA/RNA Molecule: Synthetic primer"
tacaactgugagtctggugcct

SEQ ID NO: 472 - DNA, 22 bp, Artificial Sequence
  source: /note="Description of Artificial Sequence: Synthetic primer"
  source: /note="Description of Combined DNA/RNA Molecule: Synthetic primer"
caagacagagagcugggtucca

SEQ ID NO: 473 - DNA, 22 bp, Artificial Sequence
  source: /note="Description of Artificial Sequence: Synthetic primer"
  source: /note="Description of Combined DNA/RNA Molecule: Synthetic primer"
taggauggagagtcgaguccca

SEQ ID NO: 474 - DNA, 22 bp, Artificial Sequence
  source: /note="Description of Artificial Sequence: Synthetic primer"
  source: /note="Description of Combined DNA/RNA Molecule: Synthetic primer"
tacaacggutaacctggucccc

SEQ ID NO: 475 - DNA, 23 bp, Artificial Sequence
  source: /note="Description of Artificial Sequence: Synthetic primer"
  source: /note="Description of Combined DNA/RNA Molecule: Synthetic primer"
tacaactgtgaguctggtgccut

SEQ ID NO: 476 - DNA, 23 bp, Artificial Sequence
  source: /note="Description of Artificial Sequence: Synthetic primer"
  source: /note="Description of Combined DNA/RNA Molecule: Synthetic primer"
taggauggagagtcgagucccat

SEQ ID NO: 477 - DNA, 23 bp, Artificial Sequence
  source: /note="Description of Artificial Sequence: Synthetic primer"
  source: /note="Description of Combined DNA/RNA Molecule: Synthetic primer"
tacaacagugagccaactuccct

SEQ ID NO: 478 - DNA, 23 bp, Artificial Sequence
  source: /note="Description of Artificial Sequence: Synthetic primer"
  source: /note="Description of Combined DNA/RNA Molecule: Synthetic primer"
ctacaactgugagtctggugcct

SEQ ID NO: 479 - DNA, 23 bp, Artificial Sequence
  source: /note="Description of Artificial Sequence: Synthetic primer"
  source: /note="Description of Combined DNA/RNA Molecule: Synthetic primer"
ctaggauggagagtcgaguccca

SEQ ID NO: 480 - DNA, 24 bp, Artificial Sequence
  source: /note="Description of Artificial Sequence: Synthetic primer"
  source: /note="Description of Combined DNA/RNA Molecule: Synthetic primer"
ctacaactgtgaguctggtgccut

SEQ ID NO: 481 - DNA, 24 bp, Artificial Sequence
  source: /note="Description of Artificial Sequence: Synthetic primer"
  source: /note="Description of Combined DNA/RNA Molecule: Synthetic primer"
ctaggauggagagtcgagucccat

SEQ ID NO: 482 - DNA, 24 bp, Artificial Sequence
  source: /note="Description of Artificial Sequence: Synthetic primer"
  source: /note="Description of Combined DNA/RNA Molecule: Synthetic primer"
ctacaacagugagccaactuccct

SEQ ID NO: 483 - DNA, 21 bp, Artificial Sequence
  source: /note="Description of Artificial Sequence: Synthetic primer"
aactatgttttggtatcgtca

SEQ ID NO: 484 - DNA, 24 bp, Artificial Sequence
  source: /note="Description of Artificial Sequence: Synthetic primer"
cacgatgttctggtaccgtcagca

SEQ ID NO: 485 - DNA, 22 bp, Artificial Sequence
  source: /note="Description of Artificial Sequence: Synthetic primer"
cagtgtgtcctggtaccaacag

SEQ ID NO: 486 - DNA, 21 bp, Artificial Sequence
  source: /note="Description of Artificial Sequence: Synthetic primer"
aaccctttattggtaccgaca

SEQ ID NO: 487 - DNA, 22 bp, Artificial Sequence
  source: /note="Description of Artificial Sequence: Synthetic primer"
atcccttttttggtaccaacag

SEQ ID NO: 488 - DNA, 22 bp, Artificial Sequence
  source: /note="Description of Artificial Sequence: Synthetic primer"
aaccctttattggtatcaacag

SEQ ID NO: 489 - DNA, 21 bp, Artificial Sequence
  source: /note="Description of Artificial Sequence: Synthetic primer"
cgctatgtattggtacaagca

SEQ ID NO: 490 - DNA, 25 bp, Artificial Sequence
  source: /note="Description of Artificial Sequence: Synthetic primer"
ctcccgttttctggtacagacagac

SEQ ID NO: 491 - DNA, 22 bp, Artificial Sequence
  source: /note="Description of Artificial Sequence: Synthetic primer"
cgctatgtattggtataaacag

SEQ ID NO: 492 - DNA, 26 bp, Artificial Sequence
  source: /note="Description of Artificial Sequence: Synthetic primer"
ttatgtttactggtatcgtaagaagc

SEQ ID NO: 493 - DNA, 22 bp, Artificial Sequence
  source: /note="Description of Artificial Sequence: Synthetic primer"
caaaatgtactggtatcaacaa

SEQ ID NO: 494 - DNA, 25 bp, Artificial Sequence
  source: /note="Description of Artificial Sequence: Synthetic primer"
atacatgtactggtatcgacaagac

SEQ ID NO: 495 - DNA, 23 bp, Artificial Sequence
  source: /note="Description of Artificial Sequence: Synthetic primer"
ggccatgtactggtatagacaag

SEQ ID NO: 496 - DNA, 24 bp, Artificial Sequence
  source: /note="Description of Artificial Sequence: Synthetic primer"
gtatatgtcctggtatcgacaaga

SEQ ID NO: 497 - DNA, 24 bp, Artificial Sequence
  source: /note="Description of Artificial Sequence: Synthetic primer"
taacctttattggtatcgacgtgt

SEQ ID NO: 498 - DNA, 21 bp, Artificial Sequence
  source: /note="Description of Artificial Sequence: Synthetic primer"
ggccatgtactggtaccgaca

SEQ ID NO: 499 - DNA, 22 bp, Artificial Sequence
  source: /note="Description of Artificial Sequence: Synthetic primer"
tcatgtttactggtatcggcag

SEQ ID NO: 500 - DNA, 27 bp, Artificial Sequence
  source: /note="Description of Artificial Sequence: Synthetic primer"
ttatgtttattggtatcaacagaatca

SEQ ID NO: 501 - DNA, 21 bp, Artificial Sequence
  source: /note="Description of Artificial Sequence: Synthetic primer"
caacctatactggtaccgaca

SEQ ID NO: 502 - DNA, 22 bp, Artificial Sequence
  source: /note="Description of Artificial Sequence: Synthetic primer"
taccctttactggtaccggcag

SEQ ID NO: 503 - DNA, 26 bp, Artificial Sequence
  source: /note="Description of Artificial Sequence: Synthetic primer"
atacttctattggtacagacaaatct

SEQ ID NO: 504 - DNA, 21 bp, Artificial Sequence
  source: /note="Description of Artificial Sequence: Synthetic primer"
cacggtctactggtaccagca

SEQ ID NO: 505 - DNA, 21 bp, Artificial Sequence
  source: /note="Description of Artificial Sequence: Synthetic primer"
cgtcatgtactggtaccagca